European Patent Application EP 4 748 401 A1, published May 27, 2026. Title: 一种可用于筛选针对RNA重复序列药物的报告系统. Applicant: 中国科学院上海营养与健康研究所. The sequence listing filed with the application follows.

SEQUENCE LISTING (120 sequences)

SEQ ID NO: 1 - protein, 349 aa, synthetic construct
GRSRLLEDFRNNRYPNLQLREIAGHIMEFSQDQHGSRFIELKLERATPAERQLVFNEILQAAYQLMVDVFGNYVIQKFFEFGSLEQKLALAERIRGHVLSLALQMYGSYVIRKALEFIPSDQQNEMVRELDGHVLKCVKDQNGSYVVEKCIECVQPQSLQFIIDAFKGQVFALSTHPYGNRVIQRILEHCLPDQTLPILEELHQHTEQLVQDQYGSYVIRHVLEHGRPEDKSKIVAEIRGNVLVLSQHKFASNVVEKCVTHASRTERAVLIDEVCTMNDGPHSALYTMMKDQYANYVVQKMIDVAEPGQRKIVMHKIRPHIATLRKYTYGKHILAKLEKYYMKNGVDLG

SEQ ID NO: 2 - DNA, 204 bp, synthetic construct
  source 1..204: mol_type = other DNA
gtgatgcggttttggcagtacatcaatgggcgtggatagcggtttgactcacggggatttccaagtctccaccccattgacgtcaatgggagtttgttttggcaccaaaatcaacgggactttccaaaatgtcgtaacaactccgccccattgacgcaaatgggcggtaggcgtgtacggtgggaggtctatataagcagagct

SEQ ID NO: 3 - DNA, 584 bp, synthetic construct
  source 1..584: mol_type = other DNA
gcgttacataacttacggtaaatggcccgcctggctgaccgcccaacgacccccgcccattgacgtcaataatgacgtatgttcccatagtaacgccaatagggactttccattgacgtcaatgggtggagtatttacggtaaactgcccacttggcagtacatcaagtgtatcatatgccaagtacgccccctattgacgtcaatgacggtaaatggcccgcctggcattatgcccagtacatgaccttatgggactttcctacttggcagtacatctacgtattagtcatcgctattaccatggtcgaggtgagccccacgttctgcttcactctccccatctcccccccctccccacccccaattttgtatttatttattttttaattattttgtgcagcgatgggggcggggggggggggggggcgcgcgccaggcggggcggggcggggcgaggggcggggcggggcgaggcggagaggtgcggcggcagccaatcagagcggcgcgctccgaaagtttccttttatggcgaggcggcggcggcggcggccctataaaaagcgaagcgcgcggcgggcg

SEQ ID NO: 4 - DNA, 1000 bp, synthetic construct
  source 1..1000: mol_type = other DNA
gggtaggggaggcgcttttcccaaggcagtctggagcatgcgctttagcagccccgctgggcacttggcgctacacaagtggcctctggcctcgcacacattccacatccaccggtaggcgccaaccggctccgttctttggtggccccttcgcgccaccttctactcctcccctagtcaggaagttcccccccgccccgcagctcgcgtcgtgcaggacgtgacaaatggaagtagcacgtctcactagtctcgtgcagatggacagcaccgctgagcaatggaagcgggtaggcctttggggcagcggccaatagcagctttgctccttcgctttctgggctcagaggctgggaaggggtgggtccgggggcgggctcaggggcgggctcaggggcggggcgggcgcccgaaggtcctccggaggcccggcattctgcacgcttcaaaagcgcacgtctgccgcgctgttctcctcttcctcatctccgggcctttcggggtaggggaggcgcttttcccaaggcagtctggagcatgcgctttagcagccccgctgggcacttggcgctacacaagtggcctctggcctcgcacacattccacatccaccggtaggcgccaaccggctccgttctttggtggccccttcgcgccaccttctactcctcccctagtcaggaagttcccccccgccccgcagctcgcgtcgtgcaggacgtgacaaatggaagtagcacgtctcactagtctcgtgcagatggacagcaccgctgagcaatggaagcgggtaggcctttggggcagcggccaatagcagctttgctccttcgctttctgggctcagaggctgggaaggggtgggtccgggggcgggctcaggggcgggctcaggggcggggcgggcgcccgaaggtcctccggaggcccggcattctgcacgcttcaaaagcgcacgtctgccgcgctgttctcctcttcctcatctccgggcctttcg

SEQ ID NO: 5 - DNA, 1179 bp, synthetic construct
  source 1..1179: mol_type = other DNA
ggctccggtgcccgtcagtgggcagagcgcacatcgcccacagtccccgagaagttggggggaggggtcggcaattgaaccggtgcctagagaaggtggcgcggggtaaactgggaaagtgatgtcgtgtactggctccgcctttttcccgagggtgggggagaaccgtatataagtgcagtagtcgccgtgaacgttctttttcgcaacgggtttgccgccagaacacaggtaagtgccgtgtgtggttcccgcgggcctggcctctttacgggttatggcccttgcgtgccttgaattacttccacctggctgcagtacgtgattcttgatcccgagcttcgggttggaagtgggtgggagagttcgaggccttgcgcttaaggagccccttcgcctcgtgcttgagttgaggcctggcctgggcgctggggccgccgcgtgcgaatctggtggcaccttcgcgcctgtctcgctgctttcgataagtctctagccatttaaaatttttgatgacctgctgcgacgctttttttctggcaagatagtcttgtaaatgcgggccaagatctgcacactggtatttcggtttttggggccgcgggcggcgacggggcccgtgcgtcccagcgcacatgttcggcgaggcggggcctgcgagcgcggccaccgagaatcggacgggggtagtctcaagctggccggcctgctctggtgcctggcctcgcgccgccgtgtatcgccccgccctgggcggcaaggctggcccggtcggcaccagttgcgtgagcggaaagatggccgcttcccggccctgctgcagggagctcaaaatggaggacgcggcgctcgggagagcgggcgggtgagtcacccacacaaaggaaaagggcctttccgtcctcagccgtcgcttcatgtgactccacggagtaccgggcgccgtccaggcacctcgattagttctcgagcttttggagtacgtcgtctttaggttggggggaggggttttatgcgatggagtttccccacactgagtgggtggagactgaagttaggccagcttggcacttgatgtaattctccttggaatttgccctttttgagtttggatcttggttcattctcaagcctcagacagtggttcaaagtttttttcttccatttcaggtgtcgtga

SEQ ID NO: 6 - DNA, 317 bp, synthetic construct
  source 1..317: mol_type = other DNA
ggtgtggaaagtccccaggctccccagcaggcagaagtatgcaaagcatgcatctcaattagtcagcaaccaggtgtggaaagtccccaggctccccagcaggcagaagtatgcaaagcatgcatctcaattagtcagcaaccatagtcccgcccctaactccgcccatcccgcccctaactccgcccagttccgcccattctccgccccatggctgactaattttttttatttatgcagaggccgaggccgcctcggcctctgagctattccagaagtagtgaggaggcttttttggaggcctaggcttttgcaaa

SEQ ID NO: 7 - DNA, 278 bp, synthetic construct
  source 1..278: mol_type = other DNA
tcgaggtgagccccacgttctgcttcactctccccatctcccccccctccccacccccaattttgtatttatttattttttaattattttgtgcagcgatgggggcggggggggggggggggcgcgcgccaggcggggcggggcggggcgaggggcggggcggggcgaggcggagaggtgcggcggcagccaatcagagcggcgcgctccgaaagtttccttttatggcgaggcggcggcggcggcggccctataaaaagcgaagcgcgcggcgggcg

SEQ ID NO: 8 - DNA, 753 bp, synthetic construct
  source 1..753: mol_type = other DNA
aaatgagtcttcggacctcgcgggggccgcttaagcggtggttagggtttgtctgacgcggggggagggggaaggaacgaaacactctcattcggaggcggctcggggtttggtcttggtggccacgggcacgcagaagagcgccgcgatcctcttaagcacccccccgccctccgtggaggcgggggtttggtcggcgggtggtaactggcgggccgctgactcgggcgggtcgcgcgccccagagtgtgaccttttcggtctgctcgcagacccccgggcggcgccgccgcggcggcgacgggctcgctgggtcctaggctccatggggaccgtatacgtggacaggctctggagcatccgcacgactgcggtgatattaccggagaccttctgcgggacgagccgggtcacgcggctgacgcggagcgtccgttgggcgacaaacaccaggacggggcacaggtacactatcttgtcacccggaggcgcgagggactgcaggagcttcagggagtggcgcagctgcttcatccccgtggcccgttgctcgcgtttgctggcggtgtccccggaagaaatatatttgcatgtctttagttctatgatgacacaaaccccgcccagcgtcttgtcattggcgaattcgaacacgcagatgcagtcggggcggcgcggtcccaggtccacttcgcatattaaggtgacgcgtgtggcctcgaacaccgagcgaccctgcagcgacccgcttaa

SEQ ID NO: 9 - DNA, 1210 bp, synthetic construct
  source 1..1210: mol_type = other DNA
ggcctccgcgccgggttttggcgcctcccgcgggcgcccccctcctcacggcgagcgctgccacgtcagacgaagggcgcaggagcgtcctgatccttccgcccggacgctcaggacagcggcccgctgctcataagactcggccttagaaccccagtatcagcagaaggacattttaggacgggacttgggtgactctagggcactggttttctttccagagagcggaacaggcgaggaaaagtagtcccttctcggcgattctgcggagggatctccgtggggcggtgaacgccgatgattatataaggacgcgccgggtgtggcacagctagttccgtcgcagccgggatttgggtcgcggttcttgtttgtggatcgctgtgatcgtcacttggtgagtagcgggctgctgggctggccggggctttcgtggccgccgggccgctcggtgggacggaagcgtgtggagagaccgccaagggctgtagtctgggtccgcgagcaaggttgccctgaactgggggttggggggagcgcagcaaaatggcggctgttcccgagtcttgaatggaagacgcttgtgaggcgggctgtgaggtcgttgaaacaaggtggggggcatggtgggcggcaagaacccaaggtcttgaggccttcgctaatgcgggaaagctcttattcgggtgagatgggctggggcaccatctggggaccctgacgtgaagtttgtcactgactggagaactcggtttgtcgtctgttgcgggggcggcagttatgcggtgccgttgggcagtgcacccgtacctttgggagcgcgcgccctcgtcgtgtcgtgacgtcacccgttctgttggcttataatgcagggtggggccacctgccggtaggtgtgcggtaggcttttctccgtcgcaggacgcagggttcgggcctagggtaggctctcctgaatcgacaggcgccggacctctggtgaggggagggataagtgaggcgtcagtttctttggtcggttttatgtacctatcttcttaagtagctgaagctccggttttgaactatgcgctcggggttggcgagtgtgttttgtgaagttttttaggcaccttttgaaatgtaatcatttgggtcaatatgtaattttcagtgttagactagtaaattgtccgctaaattctggccgtttttggcttttttgttagac

SEQ ID NO: 10 - DNA, 315 bp, synthetic construct
  source 1..315: mol_type = other DNA
gagtttactccctatcagtgatagagaacgtatgtcgagtttactccctatcagtgatagagaacgatgtcgagtttactccctatcagtgatagagaacgtatgtcgagtttactccctatcagtgatagagaacgtatgtcgagtttactccctatcagtgatagagaacgtatgtcgagtttatccctatcagtgatagagaacgtatgtcgagtttactccctatcagtgatagagaacgtatgtcgaggtaggcgtgtacggtgggaggcctatataagcagagctcgtttagtgaaccgtcagatcgcc

SEQ ID NO: 11 - DNA, 103 bp, synthetic construct
  source 1..103: mol_type = other DNA
cggagtactgtcctccgagcggagtactgtcctccgactcgagcggagtactgtcctccgatcggagtactgtcctccgcgaattccggagtactgtcctccg

SEQ ID NO: 12 - DNA, 41 bp, synthetic construct
  source 1..41: mol_type = other DNA
ggggggctataaaagggggtgggggcgttcgtcctcactct

SEQ ID NO: 13 - DNA, 2513 bp, synthetic construct
  source 1..2513: mol_type = other DNA
catgaatggcatcaactctgaatcaaatctttgcagatgcacctacttctcatttccactgtcacatcatttttccagatctcgctgcctgttatgtggcccacaaaccaagacacgttttatggccattaaagctggctgatcgtcgccaaacaccaaatacatatcaatatgtacattcgagaaagaagcgatcaaagaagcgtcttcgggcgagtaggagaatgcggaggagaaggagaacgagctgatctagtatctctccacaatccaatgccaactgaccaactggccatattcggagcaatttgaagccaatttccatcgcctggcgatcgctccattcttggctatatgtttttcaccgttcccggggccattttcaaagactcgtcggtaagataagattgtgtcactcgctgtctctcttcatttgtcgaagaatgctgaggaatttcgcgatgacgtcggcgagtattttgaagaatgagaataatttgtatttatacgaaaatcagttagtggaattttctacaaaaacatgttatctatagataattttgttgcaaaatatgttgactatgacaaagattgtatgtatatacctttaatgtattctcattttcttatgtatttataatggcaatgatgatactgatgatattttaagatgatgccagaccacaggctgatttctgcgtcttttgccgaacgcagtgcatgtgcggttgttgttttttggaatagtttcaattttcggactgtccgctttgatttcagtttcttggcttattcaaaaagcaaagtaaagccaaaaaagcgagatggcaataccaaatgcggcaaaacggtagtggaaggaaaggggtgcggggcagcggaaggaagggtggggcggggcgtggcggggtctgtggctgggcgcgacgtcaccgacgttggagccactcctttgaccatgtgtgcgtgtgtgtattattcgtgtctcgccactcgccggttgtttttttctttttatctcgctctctctagcgccatctcgtacgcatgctcaacgcaccgcatgttgccgtgtcctttatgcgtcattttggctcgaaataggcaattatttaaacaaagattagtcaacgaaaacgctaaaataaataagtctacaatatggttacttattgccatgtgtgtgcagccaacgatagcaacaaaagcaacaacacagtggctttccctctttcactttttgtttgcaagcgcgtgcgagcaagacggcacgaccggcaaacgcaattacgctgacaaagagcagacgaagttttggccgaaaaacatcaaggcgcctgatacgaatgcatttgcaataacaattgcgatatttaatattgtttatgaagctgtttgacttcaaaacacacaaaaaaaaaaataaaacaaattatttgaaagagaattaggaatcggacagcttatcgttacgggctaacagcacaccgagacgaaatagcttacctgacgtcacagcctctggaagaactgccgccaagcagagagagagagaaaaagagggagagcagcttagaccgcatgtgcttgtgtgtgaggcgtctctctcttcgtctcctgtttgcgcaaacgcatagactgcactgagaaaatcgattacctattttttatgaatgaatatttgcactattactattcaaaactattaagatagcaatcacattcaatagccaaatactataccacctgagcgatgcaacgaaatgatcaatttgagcaaaaatgctgcatatttaggacggcatcattatagaaatgcttcttgctgtgtacttttctctcgtctggcagctgtttcgccgttattgttaaaaccggcttaagttaggtgtgttttctacgactagtgatgcccctactagaagatgtgtgttgcacaaatgtccctgaataaccaatttgaagtgcagatagcagtaaacgtaagctaatatgaatattatttaactgtaatgttttaatatcgctggacattactaataaacccactataaacacatgtacatatgtatgttttggcatacaatgagtagttggggaaaaaatgtgtaaaagcaccgtgaccatcacagcataaagataaccagctgaagtatcgaatatgagtaacccccaaattgaatcacatgccgcaactgataggacccatggaagtacactcttcatggcgatatacaagacacacacaagcacgaacacccagttgcggaggaaattctccgtaaatgaaaacccaatcggcgaacaattcatacccatatatggtaaaagttttgaacgcgacttgagagcggagagcattgcggctgataaggttttagcgctaagcgggctttataaaacgggctgcgggaccagttttcatatcactaccgtttgagttcttgtgctgtgtggatactcctcccgacacaaagccgctccatcagccagcagtcgtctaatccagagac

SEQ ID NO: 14 - DNA, 92 bp, synthetic construct
  source 1..92: mol_type = other DNA
atcatggagataattaaaatgataaccatctcgcaaataaataagtattttactgttttcgtaacagttttgtaataaaaaaacctataaat

SEQ ID NO: 15 - DNA, 110 bp, synthetic construct
  source 1..110: mol_type = other DNA
gacctttaattcaacccaacacaatatattatagttaaataagaattattatcaaatcatttgtatattaattaaaatactatactgtaaattacattttatttacaatc

SEQ ID NO: 16 - DNA, 2578 bp, synthetic construct
  source 1..2578: mol_type = other DNA
cattatggccttaggtcacttcatctccatggggttcttcttctgattttctagaaaatgagatgggggtgcagagagcttcctcagtgacctgcccagggtcacatcagaaatgtcagagctagaacttgaactcagattactaatcttaaattccatgccttgggggcatgcaagtacgatatacagaaggagtgaactcattagggcagatgaccaatgagtttaggaaagaagagtccagggcagggtacatctacaccacccgcccagccctgggtgagtccagccacgttcacctcattatagttgcctctctccagtcctaccttgacgggaagcacaagcagaaactgggacaggagccccaggagaccaaatcttcatggtccctctgggaggatgggtggggagagctgtggcagaggcctcaggaggggccctgctgctcagtggtgacagataggggtgagaaagcagacagagtcattccgtcagcattctgggtctgtttggtacttcttctcacgctaaggtggcggtgtgatatgcacaatggctaaaaagcagggagagctggaaagaaacaaggacagagacagaggccaagtcaaccagaccaattcccagaggaagcaaagaaaccattacagagactacaagggggaagggaaggagagatgaattagcttcccctgtaaaccttagaacccagctgttgccagggcaacggggcaatacctgtctcttcagaggagatgaagttgccagggtaactacatcctgtctttctcaaggaccatcccagaatgtggcacccactagccgttaccatagcaactgcctctttgccccacttaatcccatcccgtctgttaaaagggccctatagttggaggtgggggaggtaggaagagcgatgatcacttgtggactaagtttgttcgcatccccttctccaaccccctcagtacatcaccctgggggaacagggtccacttgctcctgggcccacacagtcctgcagtattgtgtatataaggccagggcaaagaggagcaggttttaaagtgaaaggcaggcaggtgttggggaggcagttaccggggcaacgggaacagggcgtttcggaggtggttgccatggggacctggatgctgacgaaggctcgcgaggctgtgagcagccacagtgccctgctcagaagccccaagctcgtcagtcaagccggttctccgtttgcactcaggagcacgggcaggcgagtggcccctagttctgggggcagccattatggccttaggtcacttcatctccatggggttcttcttctgattttctagaaaatgagatgggggtgcagagagcttcctcagtgacctgcccagggtcacatcagaaatgtcagagctagaacttgaactcagattactaatcttaaattccatgccttgggggcatgcaagtacgatatacagaaggagtgaactcattagggcagatgaccaatgagtttaggaaagaagagtccagggcagggtacatctacaccacccgcccagccctgggtgagtccagccacgttcacctcattatagttgcctctctccagtcctaccttgacgggaagcacaagcagaaactgggacaggagccccaggagaccaaatcttcatggtccctctgggaggatgggtggggagagctgtggcagaggcctcaggaggggccctgctgctcagtggtgacagataggggtgagaaagcagacagagtcattccgtcagcattctgggtctgtttggtacttcttctcacgctaaggtggcggtgtgatatgcacaatggctaaaaagcagggagagctggaaagaaacaaggacagagacagaggccaagtcaaccagaccaattcccagaggaagcaaagaaaccattacagagactacaagggggaagggaaggagagatgaattagcttcccctgtaaaccttagaacccagctgttgccagggcaacggggcaatacctgtctcttcagaggagatgaagttgccagggtaactacatcctgtctttctcaaggaccatcccagaatgtggcacccactagccgttaccatagcaactgcctctttgccccacttaatcccatcccgtctgttaaaagggccctatagttggaggtgggggaggtaggaagagcgatgatcacttgtggactaagtttgttcgcatccccttctccaaccccctcagtacatcaccctgggggaacagggtccacttgctcctgggcccacacagtcctgcagtattgtgtatataaggccagggcaaagaggagcaggttttaaagtgaaaggcaggcaggtgttggggaggcagttaccggggcaacgggaacagggcgtttcggaggtggttgccatggggacctggatgctgacgaaggctcgcgaggctgtgagcagccacagtgccctgctcagaagccccaagctcgtcagtcaagccggttctccgtttgcactcaggagcacgggcaggcgagtggcccctagttctgggggcagc

SEQ ID NO: 17 - DNA, 114 bp, synthetic construct
  source 1..114: mol_type = other DNA
cattttgacacccccataatatttttccagaattaacagtataaattgcatctcttgttcaagagttccctatcactctctttaatcactactcacagtaacctcaactcctgc

SEQ ID NO: 18 - DNA, 229 bp, synthetic construct
  source 1..229: mol_type = other DNA
aatgtagtcttatgcaatactcttgtagtcttgcaacatggtaacgatgagttagcaacatgccttacaaggagagaaaaagcaccgtgcatgccgattggtggaagtaaggtggtacgatcgtgccttattaggaaggcaacagacgggtctgacatggattggacgaaccactgaattgccgcattgcagagatattgtatttaagtgcctagctcgatacataaac

SEQ ID NO: 19 - DNA, 442 bp, synthetic construct
  source 1..442: mol_type = other DNA
cggattagaagccgccgagcgggtgacagccctccgaaggaagactctcctccgtgcgtcctcgtcttcaccggtcgcgttcctgaaacgcagatgtgcctcgcgccgcactgctccgaacaataaagattctacaatactagcttttatggttatgaagaggaaaaattggcagtaacctggccccacaaaccttcaaatgaacgaatcaaattaacaaccataggatgataatgcgattagttttttagccttatttctggggtaattaatcagcgaagcgatgatttttgatctattaacagatatataaatgcaaaaactgcataaccactttaactaatactttcaacattttcggtttgtattacttcttattcaaatgtaataaaagtatcaacaaaaaattgttaatatacctctatactttaacgtcaaggag

SEQ ID NO: 20 - DNA, 387 bp, synthetic construct
  source 1..387: mol_type = other DNA
aatgtttctactccttttttactcttccagattttctcggactccgcgcatcgccgtaccacttcaaaacacccaagcacagcatactaaattttccctctttcttcctctagggtgtcgttaattacccgtactaaaggtttggaaaagaaaaaagagaccgcctcgtttctttttcttcgtcgaaaaaggcaataaaaatttttatcacgtttctttttcttgaaatttttttttttagtttttttctctttcagtgacctccattgatatttaagttaataaacggtcttcaatttctcaagtttcagtttcatttttcttgttctattacaactttttttacttcttgttcattagaaagaaagcatagcaatctaatctaag

SEQ ID NO: 21 - DNA, 667 bp, synthetic construct
  source 1..667: mol_type = other DNA
tcattatcaatactgccatttcaaagaatacgtaaataattaatagtagtgattttcctaactttatttagtcaaaaaattagccttttaattctgctgtaacccgtacatgcccaaaatagggggcgggttacacagaatatataacatcgtaggtgtctgggtgaacagtttattcctggcatccactaaatataatggagcccgctttttaagctggcatccagaaaaaaaaagaatcccagcaccaaaatattgttttcttcaccaaccatcagttcataggtccattctcttagcgcaactacagagaacaggggcacaaacaggcaaaaaacgggcacaacctcaatggagtgatgcaacctgcctggagtaaatgatgacacaaggcaattgacccacgcatgtatctatctcattttcttacaccttctattaccttctgctctctctgatttggaaaaagctgaaaaaaaaggttgaaaccagttccctgaaattattcccctacttgactaataagtatataaagacggtaggtattgattgtaattctgtaaatctatttcttaaacttcttaaattctacttttatagttagtcttttttttagttttaaaacaccaagaacttagtttcgaataaacacacataaacaaacaaa

SEQ ID NO: 22 - DNA, 705 bp, synthetic construct
  source 1..705: mol_type = other DNA
atccttttgttgtttccgggtgtacaatatggacttcctcttttctggcaaccaaacccatacatcgggattcctataataccttcgttggtctccctaacatgtaggtggcggaggggagatatacaatagaacagataccagacaagacataatgggctaaacaagactacaccaattacactgcctcattgatggtggtacataacgaactaatactgtagccctagacttgatagccatcatcatatcgaagtttcactaccctttttccatttgccatctattgaagtaataataggcgcatgcaacttcttttctttttttttcttttctctctcccccgttgttgtctcaccatatccgcaatgacaaaaaaatgatggaagacactaaaggaaaaaattaacgacaaagacagcaccaacagatgtcgttgttccagagctgatgaggggtatctcgaagcacacgaaactttttccttccttcattcacgcacactactctctaatgagcaacggtatacggccttccttccagttacttgaatttgaaataaaaaaaagtttgctgtcttgctatcaagtataaatagacctgcaattattaatcttttgtttcctcgtcattgttctcgttccctttcttccttgtttctttttctgcacaatatttcaagctataccaagcatacaatcaact

SEQ ID NO: 23 - DNA, 19 bp, synthetic construct
  source 1..19: mol_type = other DNA
taatacgactcactatagg

SEQ ID NO: 24 - DNA, 19 bp, synthetic construct
  source 1..19: mol_type = other DNA
aattaaccctcactaaagg

SEQ ID NO: 25 - DNA, 19 bp, synthetic construct
  source 1..19: mol_type = other DNA
atttaggtgacactataga

SEQ ID NO: 26 - DNA, 166 bp, synthetic construct
  source 1..166: mol_type = other DNA
aaagccatgacaaaaacgcgtaacaaaagtgtctataatcacggcagaaaagtccacattgattatttgcacggcgtcacactttgctatgccatagcatttttatccataagattagcggatcctacctgacgctttttatcgcaactctctactgtttctccat

SEQ ID NO: 27 - DNA, 148 bp, synthetic construct
  source 1..148: mol_type = other DNA
gtacaatcttgatccggagcttttctttttttgccgattaagaattaattcggtcgaaaaaagaaaaggagagggccaagagggagggcattggtgactattgagcacgtgagtatacgtgattaagcacacaaaggcagcttggagt

SEQ ID NO: 28 - DNA, 29 bp, synthetic construct
  source 1..29: mol_type = other DNA
ttgacaattaatcatcggctcgtataatg

SEQ ID NO: 29 - DNA, 31 bp, synthetic construct
  source 1..31: mol_type = other DNA
tttacactttatgcttccggctcgtatgttg

SEQ ID NO: 30 - DNA, 244 bp, synthetic construct
  source 1..244: mol_type = other DNA
tctcacctaccaaacaatgcccccctgcaaaaaataaattcatataaaaaacatacagataaccatctgcggtgataaattatctctggcggtgttgacataaataccactggcggtgatactgagcacatcagcaggacgcactgaccaccatgaaggtgacgctcttaaaaattaagccctgaagaagggcagcattcaaagcagaaggctttggggtgtgtgatacgaaacgaagcattgg

SEQ ID NO: 31 - DNA, 3075 bp, synthetic construct
  source 1..3075: mol_type = other DNA
atgaccatgattacggattcactggccgtcgttttacaacgtcgtgactgggaaaaccctggcgttacccaacttaatcgccttgcagcacatccccctttcgccagctggcgtaatagcgaagaggcccgcaccgatcgcccttcccaacagttgcgcagcctgaatggcgaatggcgctttgcctggtttccggcaccagaagcggtgccggaaagctggctggagtgcgatcttcctgaggccgatactgtcgtcgtcccctcaaactggcagatgcacggttacgatgcgcccatctacaccaacgtaacctatcccattacggtcaatccgccgtttgttcccacggagaatccgacgggttgttactcgctcacatttaatgttgatgaaagctggctacaggaaggccagacgcgaattatttttgatggcgttaactcggcgtttcatctgtggtgcaacgggcgctgggtcggttacggccaggacagtcgtttgccgtctgaatttgacctgagcgcatttttacgcgccggagaaaaccgcctcgcggtgatggtgctgcgttggagtgacggcagttatctggaagatcaggatatgtggcggatgagcggcattttccgtgacgtctcgttgctgcataaaccgactacacaaatcagcgatttccatgttgccactcgctttaatgatgatttcagccgcgctgtactggaggctgaagttcagatgtgcggcgagttgcgtgactacctacgggtaacagtttctttatggcagggtgaaacgcaggtcgccagcggcaccgcgcctttcggcggtgaaattatcgatgagcgtggtggttatgccgatcgcgtcacactacgtctgaacgtcgaaaacccgaaactgtggagcgccgaaatcccgaatctctatcgtgcggtggttgaactgcacaccgccgacggcacgctgattgaagcagaagcctgcgatgtcggtttccgcgaggtgcggattgaaaatggtctgctgctgctgaacggcaagccgttgctgattcgaggcgttaaccgtcacgagcatcatcctctgcatggtcaggtcatggatgagcagacgatggtgcaggatatcctgctgatgaagcagaacaactttaacgccgtgcgctgttcgcattatccgaaccatccgctgtggtacacgctgtgcgaccgctacggcctgtatgtggtggatgaagccaatattgaaacccacggcatggtgccaatgaatcgtctgaccgatgatccgcgctggctaccggcgatgagcgaacgcgtaacgcgaatggtgcagcgcgatcgtaatcacccgagtgtgatcatctggtcgctggggaatgaatcaggccacggcgctaatcacgacgcgctgtatcgctggatcaaatctgtcgatccttcccgcccggtgcagtatgaaggcggcggagccgacaccacggccaccgatattatttgcccgatgtacgcgcgcgtggatgaagaccagcccttcccggctgtgccgaaatggtccatcaaaaaatggctttcgctacctggagagacgcgcccgctgatcctttgcgaatacgcccacgcgatgggtaacagtcttggcggtttcgctaaatactggcaggcgtttcgtcagtatccccgtttacagggcggcttcgtctgggactgggtggatcagtcgctgattaaatatgatgaaaacggcaacccgtggtcggcttacggcggtgattttggcgatacgccgaacgatcgccagttctgtatgaacggtctggtctttgccgaccgcacgccgcatccagcgctgacggaagcaaaacaccagcagcagtttttccagttccgtttatccgggcaaaccatcgaagtgaccagcgaatacctgttccgtcatagcgataacgagctcctgcactggatggtggcgctggatggtaagccgctggcaagcggtgaagtgcctctggatgtcgctccacaaggtaaacagttgattgaactgcctgaactaccgcagccggagagcgccgggcaactctggctcacagtacgcgtagtgcaaccgaacgcgaccgcatggtcagaagccgggcacatcagcgcctggcagcagtggcgtctggcggaaaacctcagtgtgacgctccccgccgcgtcccacgccatcccgcatctgaccaccagcgaaatggatttttgcatcgagctgggtaataagcgttggcaatttaaccgccagtcaggctttctttcacagatgtggattggcgataaaaaacaactgctgacgccgctgcgcgatcagttcacccgtgcaccgctggataacgacattggcgtaagtgaagcgacccgcattgaccctaacgcctgggtcgaacgctggaaggcggcgggccattaccaggccgaagcagcgttgttgcagtgcacggcagatacacttgctgatgcggtgctgattacgaccgctcacgcgtggcagcatcaggggaaaaccttatttatcagccggaaaacctaccggattgatggtagtggtcaaatggcgattaccgttgatgttgaagtggcgagcgatacaccgcatccggcgcggattggcctgaactgccagctggcgcaggtagcagagcgggtaaactggctcggattagggccgcaagaaaactatcccgaccgccttactgccgcctgttttgaccgctgggatctgccattgtcagacatgtataccccgtacgtcttcccgagcgaaaacggtctgcgctgcgggacgcgcgaattgaattatggcccacaccagtggcgcggcgacttccagttcaacatcagccgctacagtcaacagcaactgatggaaaccagccatcgccatctgctgcacgcggaagaaggcacatggctgaatatcgacggtttccatatggggattggtggcgacgactcctggagcccgtcagtatcggcggaattccagctgagcgccggtcgctaccattaccagttggtctggtgtcaaaaataa

SEQ ID NO: 32 - protein, 1024 aa, synthetic construct
MTMITDSLAVVLQRRDWENPGVTQLNRLAAHPPFASWRNSEEARTDRPSQQLRSLNGEWRFAWFPAPEAVPESWLECDLPEADTVVVPSNWQMHGYDAPIYTNVTYPITVNPPFVPTENPTGCYSLTFNVDESWLQEGQTRIIFDGVNSAFHLWCNGRWVGYGQDSRLPSEFDLSAFLRAGENRLAVMVLRWSDGSYLEDQDMWRMSGIFRDVSLLHKPTTQISDFHVATRFNDDFSRAVLEAEVQMCGELRDYLRVTVSLWQGETQVASGTAPFGGEIIDERGGYADRVTLRLNVENPKLWSAEIPNLYRAVVELHTADGTLIEAEACDVGFREVRIENGLLLLNGKPLLIRGVNRHEHHPLHGQVMDEQTMVQDILLMKQNNFNAVRCSHYPNHPLWYTLCDRYGLYVVDEANIETHGMVPMNRLTDDPRWLPAMSERVTRMVQRDRNHPSVIIWSLGNESGHGANHDALYRWIKSVDPSRPVQYEGGGADTTATDIICPMYARVDEDQPFPAVPKWSIKKWLSLPGETRPLILCEYAHAMGNSLGGFAKYWQAFRQYPRLQGGFVWDWVDQSLIKYDENGNPWSAYGGDFGDTPNDRQFCMNGLVFADRTPHPALTEAKHQQQFFQFRLSGQTIEVTSEYLFRHSDNELLHWMVALDGKPLASGEVPLDVAPQGKQLIELPELPQPESAGQLWLTVRVVQPNATAWSEAGHISAWQQWRLAENLSVTLPAASHAIPHLTTSEMDFCIELGNKRWQFNRQSGFLSQMWIGDKKQLLTPLRDQFTRAPLDNDIGVSEATRIDPNAWVERWKAAGHYQAEAALLQCTADTLADAVLITTAHAWQHQGKTLFISRKTYRIDGSGQMAITVDVEVASDTPHPARIGLNCQLAQVAERVNWLGLGPQENYPDRLTAACFDRWDLPLSDMYTPYVFPSENGLRCGTRELNYGPHQWRGDFQFNISRYSQQQLMETSHRHLLHAEEGTWLNIDGFHMGIGGDDSWSPSVSAEFQLSAGRYHYQLVWCQK

SEQ ID NO: 33 - DNA, 711 bp, synthetic construct
  source 1..711: mol_type = other DNA
atggtgagcaagggcgaggaggataacatggccatcatcaaggagttcatgcgcttcaaggtgcacatggagggctccgtgaacggccacgagttcgagatcgagggcgagggcgagggccgcccctacgagggcacccagaccgccaagctgaaggtgaccaagggtggccccctgcccttcgcctgggacatcctgtcccctcagttcatgtacggctccaaggcctacgtgaagcaccccgccgacatccccgactacttgaagctgtccttccccgagggcttcaagtgggagcgcgtgatgaacttcgaggacggcggcgtggtgaccgtgacccaggactcctccctgcaggacggcgagttcatctacaaggtgaagctgcgcggcaccaacttcccctccgacggccccgtaatgcagaagaagaccatgggctgggaggcctcctccgagcggatgtaccccgaggacggcgccctgaagggcgagatcaagcagaggctgaagctgaaggacggcggccactacgacgctgaggtcaagaccacctacaaggccaagaagcccgtgcagctgcccggcgcctacaacgtcaacatcaagttggacatcacctcccacaacgaggactacaccatcgtggaacagtacgaacgcgccgagggccgccactccaccggcggcatggacgagctgtacaagtag

SEQ ID NO: 34 - protein, 236 aa, synthetic construct
MVSKGEEDNMAIIKEFMRFKVHMEGSVNGHEFEIEGEGEGRPYEGTQTAKLKVTKGGPLPFAWDILSPQFMYGSKAYVKHPADIPDYLKLSFPEGFKWERVMNFEDGGVVTVTQDSSLQDGEFIYKVKLRGTNFPSDGPVMQKKTMGWEASSERMYPEDGALKGEIKQRLKLKDGGHYDAEVKTTYKAKKPVQLPGAYNVNIKLDITSHNEDYTIVEQYERAEGRHSTGGMDELYK

SEQ ID NO: 35 - DNA, 717 bp, synthetic construct
  source 1..717: mol_type = other DNA
atgagtaaaggagaagaacttttcactggagttgtcccaattcttgttgaattagatggtgatgttaatgggcacaaattttctgtcagtggagagggtgaaggtgatgcaacatacggaaaacttacccttaaatttatttgcactactggaaaactacctgttccatggccaacacttgtcactactttctcttatggtgttcaatgcttttcaagatacccagatcatatgaaacggcatgactttttcaagagtgccatgcccgaaggttatgtacaggaaagaactatatttttcaaagatgacgggaactacaagacacgtgctgaagtcaagtttgaaggtgatacccttgttaatagaatcgagttaaaaggtattgattttaaagaagatggaaacattcttggacacaaattggaatacaactataactcacacaatgtatacatcatggcagacaaacaaaagaatggaatcaaagttaacttcaaaattagacacaacattgaagatggaagcgttcaactagcagaccattatcaacaaaatactccaattggcgatggccctgtccttttaccagacaaccattacctgtccacacaatctgccctttcgaaagatcccaacgaaaagagagaccacatggtccttcttgagtttgtaacagctgctgggattacacatggcatggatgaactatacaaatag

SEQ ID NO: 36 - protein, 238 aa, synthetic construct
MSKGEELFTGVVPILVELDGDVNGHKFSVSGEGEGDATYGKLTLKFICTTGKLPVPWPTLVTTFSYGVQCFSRYPDHMKRHDFFKSAMPEGYVQERTIFFKDDGNYKTRAEVKFEGDTLVNRIELKGIDFKEDGNILGHKLEYNYNSHNVYIMADKQKNGIKVNFKIRHNIEDGSVQLADHYQQNTPIGDGPVLLPDNHYLSTQSALSKDPNEKRDHMVLLEFVTAAGITHGMDELYK

SEQ ID NO: 37 - DNA, 720 bp, synthetic construct
  source 1..720: mol_type = other DNA
atggtgagcaagggcgaggagctgttcaccggggtggtgcccatcctggtcgagctggacggcgacgtaaacggccacaagttcagcgtgtccggcgagggcgagggcgatgccacctacggcaagctgaccctgaagttcatctgcaccaccggcaagctgcccgtgccctggcccaccctcgtgaccaccctgacctacggcgtgcagtgcttcagccgctaccccgaccacatgaagcagcacgacttcttcaagtccgccatgcccgaaggctacgtccaggagcgcaccatcttcttcaaggacgacggcaactacaagacccgcgccgaggtgaagttcgagggcgacaccctggtgaaccgcatcgagctgaagggcatcgacttcaaggaggacggcaacatcctggggcacaagctggagtacaactacaacagccacaacgtctatatcatggccgacaagcagaagaacggcatcaaggtgaacttcaagatccgccacaacatcgaggacggcagcgtgcagctcgccgaccactaccagcagaacacccccatcggcgacggccccgtgctgctgcccgacaaccactacctgagcacccagtccgccctgagcaaagaccccaacgagaagcgcgatcacatggtcctgctggagttcgtgaccgccgccgggatcactctcggcatggacgagctgtacaagtaa

SEQ ID NO: 38 - protein, 239 aa, synthetic construct
MVSKGEELFTGVVPILVELDGDVNGHKFSVSGEGEGDATYGKLTLKFICTTGKLPVPWPTLVTTLTYGVQCFSRYPDHMKQHDFFKSAMPEGYVQERTIFFKDDGNYKTRAEVKFEGDTLVNRIELKGIDFKEDGNILGHKLEYNYNSHNVYIMADKQKNGIKVNFKIRHNIEDGSVQLADHYQQNTPIGDGPVLLPDNHYLSTQSALSKDPNEKRDHMVLLEFVTAAGITLGMDELYK

SEQ ID NO: 39 - DNA, 705 bp, synthetic construct
  source 1..705: mol_type = other DNA
atggtgagcaagggcgaggaggtcatcaaagagttcatgcgcttcaaggtgcgcatggagggctccatgaacggccacgagttcgagatcgagggcgagggcgagggccgcccctacgagggcacccagaccgccaagctgaaggtgaccaagggcggccccctgcccttcgcctgggacatcctgtccccccagttcatgtacggctccaaggcgtacgtgaagcaccccgccgacatccccgattacaagaagctgtccttccccgagggcttcaagtgggagcgcgtgatgaacttcgaggacggcggtctggtgaccgtgacccaggactcctccctgcaggacggcacgctgatctacaaggtgaagatgcgcggcaccaacttcccccccgacggccccgtaatgcagaagaagaccatgggctgggaggcctccaccgagcgcctgtacccccgcgacggcgtgctgaagggcgagatccaccaggccctgaagctgaaggacggcggccactacctggtggagttcaagaccatctacatggccaagaagcccgtgcaactgcccggctactactacgtggacaccaagctggacatcacctcccacaacgaggactacaccatcgtggaacagtacgagcgctccgagggccgccaccacctgttcctgtacggcatggacgagctgtacaagtaa

SEQ ID NO: 40 - protein, 234 aa, synthetic construct
MVSKGEEVIKEFMRFKVRMEGSMNGHEFEIEGEGEGRPYEGTQTAKLKVTKGGPLPFAWDILSPQFMYGSKAYVKHPADIPDYKKLSFPEGFKWERVMNFEDGGLVTVTQDSSLQDGTLIYKVKMRGTNFPPDGPVMQKKTMGWEASTERLYPRDGVLKGEIHQALKLKDGGHYLVEFKTIYMAKKPVQLPGYYYVDTKLDITSHNEDYTIVEQYERSEGRHHLFLYGMDELYK

SEQ ID NO: 41 - DNA, 720 bp, synthetic construct
  source 1..720: mol_type = other DNA
atggtgagcaagggcgaggagctgttcaccggggtggtgcccatcctggtcgagctggacggcgacgtaaacggccacaagttcagcgtgtccggcgagggcgagggcgatgccacctacggcaagctgaccctgaagttcatctgcaccaccggcaagctgcccgtgccctggcccaccctcgtgaccaccctgagccacggcgtccagtgcttcagccgctaccccgaccacatgaagcagcacgacttcttcaagtccgccatgcccgaaggctacgtccaggagcgcaccatcttcttcaaggacgacggcaactacaagacccgcgccgaggtgaagttcgagggcgacaccctggtgaaccgcatcgagctgaagggcatcgacttcaaggaggacggcaacatcctggggcacaagctggagtacaacttcaacagccacaacgtctatatcatggccgacaagcagaagaacggcatcaaggcgaacttcaagatccgccacaacatcgaggacggcagcgtgcagctcgccgaccactaccagcagaacacccccatcggcgacggccccgtgctgctgcccgacagccactacctgagcacccagtccgccctgagcaaagaccccaacgagaagcgcgatcacatggtcctgctggagttcgtgaccgccgccgggatcactctcggcatggacgagctgtacaagtaa

SEQ ID NO: 42 - protein, 239 aa, synthetic construct
MVSKGEELFTGVVPILVELDGDVNGHKFSVSGEGEGDATYGKLTLKFICTTGKLPVPWPTLVTTLSHGVQCFSRYPDHMKQHDFFKSAMPEGYVQERTIFFKDDGNYKTRAEVKFEGDTLVNRIELKGIDFKEDGNILGHKLEYNFNSHNVYIMADKQKNGIKANFKIRHNIEDGSVQLADHYQQNTPIGDGPVLLPDSHYLSTQSALSKDPNEKRDHMVLLEFVTAAGITLGMDELYK

SEQ ID NO: 43 - DNA, 720 bp, synthetic construct
  source 1..720: mol_type = other DNA
atggtgagcaagggcgaggagctgttcaccggggtggtgcccatcctggtcgagctggacggcgacgtaaacggccacaagttcagcgtgtccggcgagggcgagggcgatgccacctacggcaagctgaccctgaagttcatctgcaccaccggcaagctgcccgtgccctggcccaccctcgtgaccaccttcggctacggcgtgcagtgcttcgcccgctaccccgaccacatgcgccagcacgacttcttcaagtccgccatgcccgaaggctacgtccaggagcgcaccatcttcttcaaggacgacggcaactacaagacccgcgccgaggtgaagttcgagggcgacaccctggtgaaccgcatcgagctgaagggcatcgacttcaaggaggacggcaacatcctggggcacaagctggagtacaactacaacagccacaacgtctatatcatggccgacaagcagaagaacggcatcaaggtgaacttcaagatccgccacaacatcgaggacggcagcgtgcagctcgccgaccactaccagcagaacacccccatcggcgacggccccgtgctgctgcccgacaaccactacctgagctaccagtccgccctgagcaaagaccccaacgagaagcgcgatcacatggtcctgctggagttcgtgaccgccgccgggatcactctcggcatggacgagctgtacaagtaa

SEQ ID NO: 44 - protein, 239 aa, synthetic construct
MVSKGEELFTGVVPILVELDGDVNGHKFSVSGEGEGDATYGKLTLKFICTTGKLPVPWPTLVTTFGYGVQCFARYPDHMRQHDFFKSAMPEGYVQERTIFFKDDGNYKTRAEVKFEGDTLVNRIELKGIDFKEDGNILGHKLEYNYNSHNVYIMADKQKNGIKVNFKIRHNIEDGSVQLADHYQQNTPIGDGPVLLPDNHYLSYQSALSKDPNEKRDHMVLLEFVTAAGITLGMDELYK

SEQ ID NO: 45 - DNA, 696 bp, synthetic construct
  source 1..696: mol_type = other DNA
atggctcagtcaaagcacggtctaacaaaagaaatgacaatgaaataccgtatggaagggtgcgtcgatggacataaatttgtgatcacgggagagggcattggatatccgttcaaagggaaacaggctattaatctgtgtgtggtcgaaggtggaccattgccatttgccgaagacatattgtcagctgcctttatgtacggaaacagggttttcactgaatatcctcaagacatagctgactatttcaagaactcgtgtcctgctggttatacatgggacaggtcttttctctttgaggatggagcagtttgcatatgtaatgcagatataacagtgagtgttgaagaaaactgcatgtatcatgagtccaaattttatggagtgaattttcctgctgatggacctgtgatgaaaaagatgacagataactgggagccatcctgcgagaagatcataccagtacctaagcaggggatattgaaaggggatgtctccatgtacctccttctgaaggatggtgggcgtttacggtgccaattcgacacagtttacaaagcaaagtctgtgccaagaaagatgccggactggcacttcatccagcataagctcacccgtgaagaccgcagcgatgctaagaatcagaaatggcatctgacagaacatgctattgcatccggatctgcattgccctga

SEQ ID NO: 46 - protein, 231 aa, synthetic construct
MAQSKHGLTKEMTMKYRMEGCVDGHKFVITGEGIGYPFKGKQAINLCVVEGGPLPFAEDILSAAFMYGNRVFTEYPQDIADYFKNSCPAGYTWDRSFLFEDGAVCICNADITVSVEENCMYHESKFYGVNFPADGPVMKKMTDNWEPSCEKIIPVPKQGILKGDVSMYLLLKDGGRLRCQFDTVYKAKSVPRKMPDWHFIQHKLTREDRSDAKNQKWHLTEHAIASGSALP

SEQ ID NO: 47 - DNA, 1653 bp, synthetic construct
  source 1..1653: mol_type = other DNA
atggaagatgccaaaaacattaagaaaggcccagcgccattctacccactcgaagacgggaccgctggcgagcagctgcataaagccatgaagcgctacgccctggtgcccggcaccatcgcctttaccgacgcacatatcgaggtggacattacctacgccgagtacttcgagatgagcgttcggctggcagaagctatgaagcgctatgggctgaatacaaaccatcggatcgtggtgtgtagcgagaatagcttgcagttcttcatgcccgtgttgggtgccctgttcatcggtgtggctgtggccccagctaacgacatctacaacgagcgcgagctgctgaacagcatgggcatcagccagcccaccgtcgtattcgtgagcaagaaagggctgcaaaagatcctcaacgtgcaaaagaagctaccgatcatacaaaagatcatcatcatggatagcaagaccgactaccagggcttccaaagcatgtacaccttcgtgacttcccatttgccacccggcttcaacgagtacgacttcgtgcccgagagcttcgaccgggacaaaaccatcgccctgatcatgaacagtagtggcagtaccggattgcccaagggcgtagccctaccgcaccgcaccgcttgtgtccgattcagtcatgcccgcgaccccatcttcggcaaccagatcatccccgacaccgctatcctgagcgtggtgccatttcaccacggcttcggcatgttcaccacgctgggctacttgatctgcggctttcgggtcgtgctcatgtaccgcttcgaggaagagctattcttgcgcagcttgcaagactataagattcaatctgccctgctggtgcccacactatttagcttcttcgctaagagcactctcatcgacaagtacgacctaagcaacttgcacgagatcgccagcggcggggcgccgctcagcaaggaggtaggtgaggccgtggccaaacgcttccacctaccaggcatccgccagggctacggcctgacagaaacaaccagcgccattctgatcacccccgaaggggacgacaagcctggcgcagtaggcaaggtggtgcccttcttcgaggctaaggtggtggacttggacaccggtaagacactgggtgtgaaccagcgcggcgagctgtgcgtccgtggccccatgatcatgagcggctacgttaacaaccccgaggctacaaacgctctcatcgacaaggacggctggctgcatagcggcgacatcgcctactgggacgaggacgagcacttcttcatcgtggaccggctgaagagcctgatcaaatacaagggctaccaggtagccccagccgaactggagagcatcctgctgcaacaccccaacatcttcgacgccggggtcgccggcctgcccgacgacgatgccggcgagctgcccgccgcagtcgtcgtgctggaacacggtaaaaccatgaccgagaaggagatcgtggactatgtggccagccaggttacaaccgccaagaagctgcgcggtggtgttgtgttcgtggacgaggtgcctaaaggactgaccggcaagttggacgcccgcaagatccgcgagattctcattaaggccaagaagggcggcaagatcgccgtctag

SEQ ID NO: 48 - protein, 550 aa, synthetic construct
MEDAKNIKKGPAPFYPLEDGTAGEQLHKAMKRYALVPGTIAFTDAHIEVDITYAEYFEMSVRLAEAMKRYGLNTNHRIVVCSENSLQFFMPVLGALFIGVAVAPANDIYNERELLNSMGISQPTVVFVSKKGLQKILNVQKKLPIIQKIIIMDSKTDYQGFQSMYTFVTSHLPPGFNEYDFVPESFDRDKTIALIMNSSGSTGLPKGVALPHRTACVRFSHARDPIFGNQIIPDTAILSVVPFHHGFGMFTTLGYLICGFRVVLMYRFEEELFLRSLQDYKIQSALLVPTLFSFFAKSTLIDKYDLSNLHEIASGGAPLSKEVGEAVAKRFHLPGIRQGYGLTETTSAILITPEGDDKPGAVGKVVPFFEAKVVDLDTGKTLGVNQRGELCVRGPMIMSGYVNNPEATNALIDKDGWLHSGDIAYWDEDEHFFIVDRLKSLIKYKGYQVAPAELESILLQHPNIFDAGVAGLPDDDAGELPAAVVVLEHGKTMTEKEIVDYVASQVTTAKKLRGGVVFVDEVPKGLTGKLDARKIREILIKAKKGGKIAV

SEQ ID NO: 49 - DNA, 939 bp, synthetic construct
  source 1..939: mol_type = other DNA
atgaccagcaaagtgtatgatccggaacagcgcaaacgcatgattaccggcccgcagtggtgggcgcgctgcaaacagatgaacgtgctggatagctttattaactattatgatagcgaaaaacatgcggaaaacgcggtgatttttctgcatggcaacgcggcgagcagctatctgtggcggcatgtggtgccgcatattgaaccagtggcgcgctgcattattccggatctgattggcatgggcaaaagcggcaaaagcggcaacggcagctatcgcctgctggatcattataaatatctgaccgcgtggtttgaactgctgaacctgccgaaaaaaattatttttgtgggccatgattggggcgcgtgcctggcgtttcattatagctatgaacatcaggataaaattaaagcgattgtgcacgcggaaagcgtggtggatgtgattgaaagctgggatgaatggccggatattgaagaagatattgcgctgattaaaagcgaagaaggcgaaaaaatggtgctggaaaacaacttttttgtggaaaccatgctgccgagcaaaattatgcgcaaactggaaccggaagaatttgcggcgtatctggaaccgtttaaagaaaaaggcgaagtgcgccgcccgaccctgagctggccgcgcgaaattccgctggtgaaaggcggcaaaccggatgtggtccagattgtgcgcaactataacgcgtatctgcgcgcgagcgatgatctgccgaaaatgtttattgaaagcgatccgggcttttttagcaacgcgattgtggaaggcgcgaaaaaatttccgaacaccgaatttgtgaaagtgaagggcctgcattttagccaggaagatgcgccggatgaaatgggcaaatatattaagagctttgtggaacgcgtgctgaaaaacgaacagggctag

SEQ ID NO: 50 - protein, 312 aa, synthetic construct
MTSKVYDPEQRKRMITGPQWWARCKQMNVLDSFINYYDSEKHAENAVIFLHGNAASSYLWRHVVPHIEPVARCIIPDLIGMGKSGKSGNGSYRLLDHYKYLTAWFELLNLPKKIIFVGHDWGACLAFHYSYEHQDKIKAIVHAESVVDVIESWDEWPDIEEDIALIKSEEGEKMVLENNFFVETMLPSKIMRKLEPEEFAAYLEPFKEKGEVRRPTLSWPREIPLVKGGKPDVVQIVRNYNAYLRASDDLPKMFIESDPGFFSNAIVEGAKKFPNTEFVKVKGLHFSQEDAPDEMGKYIKSFVERVLKNEQG

SEQ ID NO: 51 - DNA, 558 bp, synthetic construct
  source 1..558: mol_type = other DNA
atgggagtcaaagttctgtttgccctgatctgcatcgctgtggccgaggccaagcccaccgagaacaacgaagacttcaacatcgtggccgtggccagcaacttcgcgaccacggatctcgatgctgaccgcgggaagttgcccggcaagaagctgccgctggaggtgctcaaagagatggaagccaatgcccggaaagctggctgcaccaggggctgtctgatctgcctgtcccacatcaagtgcacgcccaagatgaagaagttcatcccaggacgctgccacacctacgaaggcgacaaagagtccgcacagggcggcataggcgaggcgatcgtcgacattcctgagattcctgggttcaaggacttggagcccatggagcagttcatcgcacaggtcgatctgtgtgtggactgcacaactggctgcctcaaagggcttgccaacgtgcagtgttctgacctgctcaagaagtggctgccgcaacgctgtgcgacctttgccagcaagatccagggccaggtggacaagatcaagggggccggtggtgactaa

SEQ ID NO: 52 - protein, 185 aa, synthetic construct
MGVKVLFALICIAVAEAKPTENNEDFNIVAVASNFATTDLDADRGKLPGKKLPLEVLKEMEANARKAGCTRGCLICLSHIKCTPKMKKFIPGRCHTYEGDKESAQGGIGEAIVDIPEIPGFKDLEPMEQFIAQVDLCVDCTTGCLKGLANVQCSDLLKKWLPQRCATFASKIQGQVDKIKGAGGD

SEQ ID NO: 53 - DNA, 516 bp, synthetic construct
  source 1..516: mol_type = other DNA
atggtcttcacactcgaagatttcgttggggactggcgacagacagccggctacaacctggaccaagtccttgaacagggaggtgtgtccagtttgtttcagaatctcggggtgtccgtaactccgatccaaaggattgtcctgagcggtgaaaatgggctgaagatcgacatccatgtcatcatcccgtatgaaggtctgagcggcgaccaaatgggccagatcgaaaaaatttttaaggtggtgtaccctgtggatgatcatcactttaaggtgatcctgcactatggcacactggtaatcgacggggttacgccgaacatgatcgactatttcggacggccgtatgaaggcatcgccgtgttcgacggcaaaaagatcactgtaacagggaccctgtggaacggcaacaaaattatcgacgagcgcctgatcaaccccgacggctccctgctgttccgagtaaccatcaacggagtgaccggctggcggctgtgcgaacgcattctggcgtaa

SEQ ID NO: 54 - protein, 171 aa, synthetic construct
MVFTLEDFVGDWRQTAGYNLDQVLEQGGVSSLFQNLGVSVTPIQRIVLSGENGLKIDIHVIIPYEGLSGDQMGQIEKIFKVVYPVDDHHFKVILHYGTLVIDGVTPNMIDYFGRPYEGIAVFDGKKITVTGTLWNGNKIIDERLINPDGSLLFRVTINGVTGWRLCERILA

SEQ ID NO: 55 - DNA, 1662 bp, synthetic construct
  source 1..1662: mol_type = other DNA
atgaagaccttaattcttgccgttgcattagtctactgcgccactgttcattgccaggactgtccttacgaacctgatccaccaaacacagttccaacttcctgtgaagctaaagaaggagaatgtattgatagcagctgtggcacctgcacgagagacatactatcagatggactgtgtgaaaataaaccaggaaaaacatgttgccgaatgtgtcagtatgtaattgaatgcagagtagaggccgcaggatggtttagaacattctatggaaagagattccagttccaggaacctggtacatacgtgttgggtcaaggaaccaagggcggcgactggaaggtgtccatcaccctggagaacctggatggaaccaagggggctgtgctgaccaagacaagactggaagtggctggagacatcattgacatcgctcaagctactgagaatcccatcactgtaaacggtggagctgaccctatcatcgccaacccgtacaccatcggcgaggtcaccatcgctgttgttgagatgccaggcttcaacatcaccgtcattgagttcttcaaactgatcgtgatcgacatcctcggaggaagatctgtaagaatcgccccagacacagcaaacaaaggaatgatctctggcctctgtggagatcttaaaatgatggaagatacagacttcacttcagatccagaacaactcgctattcagcctaagatcaaccaggagtttgacggttgtccactctatggaaatcctgatgacgttgcatactgcaaaggtcttctggagccgtacaaggacagctgccgcaaccccatcaacttctactactacaccatctcctgcgccttcgcccgctgtatgggtggagacgagcgagcctcacacgtgctgcttgactacagggagacgtgcgctgctcccgaaactagaggaacctgcgttttgtctggacatactttctacgatacatttgacaaagcaagataccaattccagggtccctgcaaggagattcttatggccgccgactgtttctggaacacttgggatgtgaaggtttcacacaggaatgttgactcttacactgaagtagagaaagtacgaatcaggaaacaatcgactgtagtagaactcattgttgatggaaaacagattctggttggaggagaagccgtgtccgtcccgtacagctctcagaacacttccatctactggcaagatggtgacatactgactacagccatcctacctgaagctctggtggtcaagttcaacttcaagcaactgctcgtcgtacatattagagatccattcgatggtaagacttgcggtatttgcggtaactacaaccaggatttcagtgatgattcttttgatgctgaaggagcctgtgatctgacccccaacccaccgggatgcaccgaagaacagaaacctgaagctgaacgactctgcaatagtctcttcgccggtcaaagtgatcttgatcagaaatgtaacgtgtgccacaagcctgaccgtgtcgaacgatgcatgtacgagtattgcctgaggggacaacagggtttctgtgaccacgcatgggagttcaagaaagaatgctacataaagcatggagacaccctagaagtaccagatgaatgcaaatag

SEQ ID NO: 56 - protein, 553 aa, synthetic construct
MKTLILAVALVYCATVHCQDCPYEPDPPNTVPTSCEAKEGECIDSSCGTCTRDILSDGLCENKPGKTCCRMCQYVIECRVEAAGWFRTFYGKRFQFQEPGTYVLGQGTKGGDWKVSITLENLDGTKGAVLTKTRLEVAGDIIDIAQATENPITVNGGADPIIANPYTIGEVTIAVVEMPGFNITVIEFFKLIVIDILGGRSVRIAPDTANKGMISGLCGDLKMMEDTDFTSDPEQLAIQPKINQEFDGCPLYGNPDDVAYCKGLLEPYKDSCRNPINFYYYTISCAFARCMGGDERASHVLLDYRETCAAPETRGTCVLSGHTFYDTFDKARYQFQGPCKEILMAADCFWNTWDVKVSHRNVDSYTEVEKVRIRKQSTVVELIVDGKQILVGGEAVSVPYSSQNTSIYWQDGDILTTAILPEALVVKFNFKQLLVVHIRDPFDGKTCGICGNYNQDFSDDSFDAEGACDLTPNPPGCTEEQKPEAERLCNSLFAGQSDLDQKCNVCHKPDRVERCMYEYCLRGQQGFCDHAWEFKKECYIKHGDTLEVPDECK

SEQ ID NO: 57 - DNA, 175 bp, synthetic construct
  source 1..175: mol_type = other DNA
tttctccataataatgtgtgagtagttcccagataagggaattagggttcctatagggtttcgctcatgtgttgagcatataagaaacccttagtatgtatttgtatttgtaaaatacttctatcaataaaatttctaattcctaaaaccaaaatccagtactaaaatccagatc

SEQ ID NO: 58 - DNA, 573 bp, synthetic construct
  source 1..573: mol_type = other DNA
attatccctaatacctgccaccccactcttaatcagtggtggaagaacggtctcagaactgtttgtttcaattggccatttaagtttagtagtaaaagactggttaatgataacaatgcatcgtaaaaccttcagaaggaaaggagaatgttttgtggaccactttggttttcttttttgcgtgtggcagttttaagttattagtttttaaaatcagtactttttaatggaaacaacttgaccaaaaatttgtcacagaattttgagacccattaaaaaagttaaatgagaaacctgtgtgttcctttggtcaacaccgagacatttaggtgaaagacatctaattctggttttacgaatctggaaacttcttgaaaatgtaattcttgagttaacacttctgggtggagaatagggttgttttccccccacataattggaaggggaaggaatatcatttaaagctatgggagggtttctttgattacaacactggagagaaatgcagcatgttgctgattgcctgtcactaaaacaggccaaaaactgagtccttgggttgcatagaaagct

SEQ ID NO: 59 - DNA, 112 bp, synthetic construct
  source 1..112: mol_type = other DNA
ctgtgccttctagttgccagccatctgttgtttgcccctcccccgtgccttccttgaccctggaaggtgccactcccactgtcctttcctaataaaatgaggaaattgcatc

SEQ ID NO: 60 - DNA, 477 bp, synthetic construct
  source 1..477: mol_type = other DNA
gggtggcatccctgtgacccctccccagtgcctctcctggccctggaagttgccactccagtgcccaccagccttgtcctaataaaattaagttgcatcattttgtctgactaggtgtccttctataatattatggggtggaggggggtggtatggagcaaggggcaagttgggaagacaacctgtagggcctgcggggtctattgggaaccaagctggagtgcagtggcacaatcttggctcactgcaatctccgcctcctgggttcaagcgattctcctgcctcagcctcccgagttgttgggattccaggcatgcatgaccaggctcagctaatttttgtttttttggtagagacggggtttcaccatattggccaggctggtctccaactcctaatctcaggtgatctacccaccttggcctcccaaattgctgggattacaggcgtgaaccactgctcccttccctgtcctt

SEQ ID NO: 61 - DNA, 122 bp, synthetic construct
  source 1..122: mol_type = other DNA
aacttgtttattgcagcttataatggttacaaataaagcaatagcatcacaaatttcacaaataaagcatttttttcactgcattctagttgtggtttgtccaaactcatcaatgtatctta

SEQ ID NO: 62 - DNA, 395 bp, synthetic construct
  source 1..395: mol_type = other DNA
gctcgctttcttgctgtccaatttctattaaaggttcctttgttccctaagtccaactactaaactgggggatattatgaagggccttgagcatctggattctgcctaataaaaaacatttattttcattgcaatgatgtatttaaattatttctgaatattttactaaaaagggaatgtgggaggtcagtgcatttaaaacataaagaaatgaagagctagttcaaaccttgggaaaatacactatatcttaaactccatgaaagaaggtgaggctgcaaacagctaatgcacattggcaacagcccctgatgcctatgccttattcatccctcagaaaaggattcaagtagaggcttgatttggaggttaaagttttgctatgctgtatttta

SEQ ID NO: 63 - DNA, 21 bp, synthetic construct
  source 1..21: mol_type = other DNA
ccaaaaaagaagagaaaggta

SEQ ID NO: 64 - protein, 7 aa, synthetic construct
PKKKRKV

SEQ ID NO: 65 - DNA, 108 bp, synthetic construct
  source 1..108: mol_type = other DNA
atgctgtttaatctgaggatcctgttaaacaatgcagcttttagaaatggtcacaacttcatggttcgaaattttcggtgtggacaaccactacaaaataaagtgcag

SEQ ID NO: 66 - protein, 36 aa, synthetic construct
MLFNLRILLNNAAFRNGHNFMVRNFRCGQPLQNKVQ

SEQ ID NO: 67 - DNA, 27 bp, synthetic construct
  source 1..27: mol_type = other DNA
ctgccccccctggagcggctgaccctg

SEQ ID NO: 68 - protein, 9 aa, synthetic construct
LPPLERLTL

SEQ ID NO: 69 - DNA, 441 bp, synthetic construct
  source 1..441: mol_type = other DNA
atggtgatgggcctgggcgttttgttgttggtcttcgtgctgggtctgggtctgaccccaccgaccctggctcaggataactccaggtacacacacttcctgacccagcactatgatgccaaaccacagggccgggatgacagatactgtgaaagcatcatgaggagacggggcctgacctcaccctgcaaagacatcaacacatttattcatggcaacaagcgcagcatcaaggccatctgtgaaaacaagaatggaaaccctcacagagaaaacctaagaataagcaagtcttctttccaggtcaccacttgcaagctacatggaggttccccctggcctccatgccagtaccgagccacagcggggttcagaaacgttgttgttgcttgtgaaaatggcttacctgtccacttggatcagtcaattttccgtcgtccg

SEQ ID NO: 70 - protein, 147 aa, synthetic construct
MVMGLGVLLLVFVLGLGLTPPTLAQDNSRYTHFLTQHYDAKPQGRDDRYCESIMRRRGLTSPCKDINTFIHGNKRSIKAICENKNGNPHRENLRISKSSFQVTTCKLHGGSPWPPCQYRATAGFRNVVVACENGLPVHLDQSIFRRP

SEQ ID NO: 71 - DNA, 369 bp, synthetic construct
  source 1..369: mol_type = other DNA
caggataactccaggtacacacacttcctgacccagcactatgatgccaaaccacagggccgggatgacagatactgtgaaagcatcatgaggagacggggcctgacctcaccctgcaaagacatcaacacatttattcatggcaacaagcgcagcatcaaggccatctgtgaaaacaagaatggaaaccctcacagagaaaacctaagaataagcaagtcttctttccaggtcaccacttgcaagctacatggaggttccccctggcctccatgccagtaccgagccacagcggggttcagaaacgttgttgttgcttgtgaaaatggcttacctgtccacttggatcagtcaattttccgtcgtccg

SEQ ID NO: 72 - protein, 123 aa, synthetic construct [sequence omitted]

SEQ ID NO: 73 - DNA, 1077 bp, synthetic construct
  source 1..1077: mol_type = other DNA
attgatgaaaaatacaaaattgctgatacttcagaaggaggcatctacctggggttctatgagaagcaagaagtagctgtgaagacgttctgtgagggcagcccacgtgcacagcgggaagtctcttgtctgcaaagcagccgagagaacagtcacttggtgacattctatgggagtgagagccacaggggccacttgtttgtgtgtgtcaccctctgtgagcagactctggaagcgtgtttggatgtgcacagaggggaagatgtggaaaatgaggaagatgaatttgcccgaaatgtcctgtcatctatatttaaggctgttcaagaactacacttgtcctgtggatacacccaccaggatctgcaaccacaaaacatcttaatagattctaagaaagctgctcacctggcagattttgataagagcatcaagtgggctggagatccacaggaagtcaagagagatctagaggaccttggacggctggtcctctatgtggtaaagaagggaagcatctcatttgaggatctgaaagctcaaagtaatgaagaggtggttcaactttctccagatgaggaaactaaggacctcattcatcgtctcttccatcctggggaacatgtgagggactgtctgagtgacctgctgggtcatcccttcttttggacttgggagagccgctataggacgcttcggaatgtgggaaatgaatccgacatcaaaacacgaaaatctgaaagtgagatcctcagactactgcaacctgggccttctgaacattccaaaagttttgacaagtggacgactaagattaatgaatgtgttatgaaaaaaatgaataagttttatgaaaaaagaggcaatttctaccagaacactgtgggtgatctgctaaagttcatccggaatttgggagaacacattgatgaagaaaagcataaaaagatgaaattaaaaattggagacccttccctgtattttcagaagacatttccagatctggtgatctatgtctacacaaaactacagaacacagaatatagaaagcatttcccccaaacccacagtccaaac

SEQ ID NO: 74 - protein, 359 aa, synthetic construct
IDEKYKIADTSEGGIYLGFYEKQEVAVKTFCEGSPRAQREVSCLQSSRENSHLVTFYGSESHRGHLFVCVTLCEQTLEACLDVHRGEDVENEEDEFARNVLSSIFKAVQELHLSCGYTHQDLQPQNILIDSKKAAHLADFDKSIKWAGDPQEVKRDLEDLGRLVLYVVKKGSISFEDLKAQSNEEVVQLSPDEETKDLIHRLFHPGEHVRDCLSDLLGHPFFWTWESRYRTLRNVGNESDIKTRKSESEILRLLQPGPSEHSKSFDKWTTKINECVMKKMNKFYEKRGNFYQNTVGDLLKFIRNLGEHIDEEKHKKMKLKIGDPSLYFQKTFPDLVIYVYTKLQNTEYRKHFPQTHSPN

SEQ ID NO: 75 - DNA, 357 bp, synthetic construct
  source 1..357: mol_type = other DNA
cactacttgctgcccgacactaatgtgttactgcaccagattgatgttcttgaggaccctgccatcaggaatgtaattgtgctacaaacagttcttcaagaagtgagaaatcgcagtgcccccgtatataaacgcatccgagatgtgactaataaccaagagaagcatttctatactttcactaatgagcaccatagagaaacctatgtagaacaagaacagggagaaaatgctaatgacaggaatgatagagcgattcgagtagcagcaaaatggtacaatgaacatttgaaaaaaatgtcagcagacaaccagctgcaagttatcttcataacaaatgacaggagaaacaaagag

SEQ ID NO: 76 - protein, 119 aa, synthetic construct
HYLLPDTNVLLHQIDVLEDPAIRNVIVLQTVLQEVRNRSAPVYKRIRDVTNNQEKHFYTFTNEHHRETYVEQEQGENANDRNDRAIRVAAKWYNEHLKKMSADNQLQVIFITNDRRNKE

SEQ ID NO: 77 - DNA, 384 bp, synthetic construct
  source 1..384: mol_type = other DNA
aaggaatcccgggccaagaaattccagcggcagcatatggactcagacagttcccccagcagcagctccacctactgtaaccaaatgatgaggcgccggaatatgacacaggggcggtgcaaaccagtgaacacctttgtgcacgagcccctggtagatgtccagaatgtctgtttccaggaaaaggtcacctgcaagaacgggcagggcaactgctacaagagcaactccagcatgcacatcacagactgccgcctgacaaacggctccaggtaccccaactgtgcataccggaccagcccgaaggagagacacatcattgtggcctgtgaagggagcccatatgtgccagtccactttgatgcttctgtggaggactctacc

SEQ ID NO: 78 - protein, 128 aa, synthetic construct
KESRAKKFQRQHMDSDSSPSSSSTYCNQMMRRRNMTQGRCKPVNTFVHEPLVDVQNVCFQEKVTCKNGQGNCYKSNSSMHITDCRLTNGSRYPNCAYRTSPKERHIIVACEGSPYVPVHFDASVEDST

SEQ ID NO: 79 - DNA, 1677 bp, synthetic construct
  source 1..1677: mol_type = other DNA
gctgtggccgtggacttaggcaacaggaaattagaaatatcttctggaaagctggccagatttgcagatggctctgctgtagtacagtcaggtgacactgcagtaatggtcacagcggtcagtaaaacaaaaccttccccttcccagtttatgcctttggtggttgactacagacaaaaagctgctgcagcaggtagaattcccacaaactatctgagaagagagattggtacttctgataaagaaattctaacaagtcgaataatagatcgttcaattagaccgctctttccagctggctacttctatgatacacaggttctgtgtaatctgttagcagtagatggtgtaaatgagcctgatgtcctagcaattaatggcgcttccgtagccctctcattatcagatattccttggaatggacctgttggggcagtacgaataggaataattgatggagaatatgttgttaacccaacaagaaaagaaatgtcttctagtactttaaatttagtggttgctggagcacctaaaagtcagattgtcatgttggaagcctctgcagagaacattttacagcaggacttttgccatgctatcaaagtgggagtgaaatatacccaacaaataattcagggcattcagcagttggtaaaagaaactggtgttaccaagaggacacctcagaagttatttaccccttcgccagagattgtgaaatatactcataaacttgctatggagagactctatgcagtttttacagattacgagcatgacaaagtttccagagatgaagctgttaacaaaataagattagatacggaggaacaactaaaagaaaaatttccagaagccgatccatatgaaataatagaatccttcaatgttgttgcaaaggaagtttttagaagtattgttttgaatgaatacaaaaggtgcgatggtcgggatttgacttcacttaggaatgtaagttgtgaggtagatatgtttaaaacccttcatggatcagcattatttcaaagaggacaaacacaggtgctttgtaccgttacatttgattcattagaatctggtattaagtcagatcaagttataacagctataaatgggataaaagataaaaatttcatgctgcactacgagtttcctccttatgcaactaatgaaattggcaaagtcactggtttaaatagaagagaacttgggcatggtgctcttgctgagaaagctttgtatcctgttattccccgagattttcctttcaccataagagttacatctgaagtcctagagtcaaatgggtcatcttctatggcatctgcatgtggcggaagtttagcattaatggattcaggggttccaatttcatctgctgttgcaggcgtagcaataggattggtcaccaaaaccgatcctgagaagggtgaaatagaagattatcgtttgctgacagatattttgggaattgaagattacaatggtgacatggacttcaaaatagctggcactaataaaggaataactgcattacaggctgatattaaattacctggaataccaataaaaattgtgatggaggctattcaacaagcttcagtggcaaaaaaggagatattacagatcatgaacaaaactatttcaaaacctcgagcatctagaaaagaaaatgga

SEQ ID NO: 80 - protein, 559 aa, synthetic construct
AVAVDLGNRKLEISSGKLARFADGSAVVQSGDTAVMVTAVSKTKPSPSQFMPLVVDYRQKAAAAGRIPTNYLRREIGTSDKEILTSRIIDRSIRPLFPAGYFYDTQVLCNLLAVDGVNEPDVLAINGASVALSLSDIPWNGPVGAVRIGIIDGEYVVNPTRKEMSSSTLNLVVAGAPKSQIVMLEASAENILQQDFCHAIKVGVKYTQQIIQGIQQLVKETGVTKRTPQKLFTPSPEIVKYTHKLAMERLYAVFTDYEHDKVSRDEAVNKIRLDTEEQLKEKFPEADPYEIIESFNVVAKEVFRSIVLNEYKRCDGRDLTSLRNVSCEVDMFKTLHGSALFQRGQTQVLCTVTFDSLESGIKSDQVITAINGIKDKNFMLHYEFPPYATNEIGKVTGLNRRELGHGALAEKALYPVIPRDFPFTIRVTSEVLESNGSSSMASACGGSLALMDSGVPISSAVAGVAIGLVTKTDPEKGEIEDYRLLTDILGIEDYNGDMDFKIAGTNKGITALQADIKLPGIPIKIVMEAIQQASVAKKEILQIMNKTISKPRASRKENG

SEQ ID NO: 81 - DNA, 495 bp, synthetic construct
  source 1..495: mol_type = other DNA
atggtctgggtggacctggagatgacaggattggacattgagaaggaccagattattgagatggcctgtctgataactgactctgatctcaacattttggctgaaggtcctaacctgattataaaacaaccagatgagttgctggacagcatgtcagattggtgtaaggagcatcacgggaagtctggccttaccaaggcagtgaaggagagtacaattacattgcagcaggcagagtatgaatttctgtcctttgtacgacagcagactcctccagggctctgtccacttgcaggaaattcagttcatgaagataagaagtttcttgacaaatacatgccccagttcatgaaacatcttcattatagaataattgatgtgagcactgttaaagaactgtgcagacgctggtatccagaagaatatgaatttgcaccaaagaaggctgcttctcatagggcacttgatgacattagtgaaagcatcaaagagctt

SEQ ID NO: 82 - protein, 165 aa, synthetic construct
MVWVDLEMTGLDIEKDQIIEMACLITDSDLNILAEGPNLIIKQPDELLDSMSDWCKEHHGKSGLTKAVKESTITLQQAEYEFLSFVRQQTPPGLCPLAGNSVHEDKKFLDKYMPQFMKHLHYRIIDVSTVKELCRRWYPEEYEFAPKKAASHRALDDISESIKEL

SEQ ID NO: 83 - DNA, 429 bp, synthetic construct
  source 1..429: mol_type = other DNA
gatcttctcaaaactgcatttgttaatagctgctatattaaaagtgaggaggccaaacgccaacaacttgggatagagaaagaagctgttcttctgaatcttaaaagtaatcaagaactatccgaacaagggacatctttttcacagacttgccttacacagtttcttgaagacgagtacccagacatgcccactgaaggcataaaaaatcttgttgactttctcactggtgaggaagtcgtgtgtcacgtggctagaaacttggctgtggagcagttaacactgagtgaagaattcccagtgcccccagctgtgttacagcagactttctttgcagttattggagccctgttacagagcagtggacctgagaggactgcacttttcatcagggacttcttaattactcaaatgactggaaaagagctc

SEQ ID NO: 84 - protein, 143 aa, synthetic construct
DLLKTAFVNSCYIKSEEAKRQQLGIEKEAVLLNLKSNQELSEQGTSFSQTCLTQFLEDEYPDMPTEGIKNLVDFLTGEEVVCHVARNLAVEQLTLSEEFPVPPAVLQQTFFAVIGALLQSSGPERTALFIRDFLITQMTGKEL

SEQ ID NO: 85 - DNA, 864 bp, synthetic construct
  source 1..864: mol_type = other DNA
atggctgctgtactgcagcgcgtcgagcggctgtccaatcgagtcgtgcgtgtgttgggctgtaacccgggtcccatgaccctccaaggcaccaacacctacctagtggggaccggccccaggagaatcctcattgacactggagaaccagcaattccagaatacatcagctgtttaaagcaggctctaactgaatttaacacagcaatccaggaaattgtagtgactcactggcaccgagatcattctggaggcataggagatatttgtaaaagcatcaataatgacactacctattgcattaaaaaactcccacggaatcctcagagagaagaaattataggaaatggagagcaacaatatgtttatctgaaagatggagatgtgattaagactgagggagccactctaagagttctatatacccctggccacactgatgatcacatggctctactcttagaagaggaaaatgctatcttttctggagattgcatcctaggggaaggaacaacggtatttgaagacctctatgattatatgaactctttaaaagagttattgaaaatcaaagctgatattatatatccaggacatggcccagtaattcataatgctgaagctaaaattcaacaatacatttctcacagaaatattcgagagcagcaaattcttacattatttcgtgagaactttgagaaatcatttacagtaatggagcttgtaaaaattatttacaagaatactcctgagaatttacatgaaatggctaaacataatctcttacttcatttgaaaaaactagaaaaagaaggaaaaatatttagcaacacagatcctgacaagaaatggaaagctcatctt

SEQ ID NO: 86 - protein, 288 aa, synthetic construct
MAAVLQRVERLSNRVVRVLGCNPGPMTLQGTNTYLVGTGPRRILIDTGEPAIPEYISCLKQALTEFNTAIQEIVVTHWHRDHSGGIGDICKSINNDTTYCIKKLPRNPQREEIIGNGEQQYVYLKDGDVIKTEGATLRVLYTPGHTDDHMALLLEEENAIFSGDCILGEGTTVFEDLYDYMNSLKELLKIKADIIYPGHGPVIHNAEAKIQQYISHRNIREQQILTLFRENFEKSFTVMELVKIIYKNTPENLHEMAKHNLLLHLKKLEKEGKIFSNTDPDKKWKAHL

SEQ ID NO: 87 - DNA, 513 bp, synthetic construct
  source 1..513: mol_type = other DNA
atggaggagcgcggcgattccgagccgacccccggctgcagcggcctgggtccgggcggtgttcgcggctttggcgacggcggtggagctccttcgtgggcccctgaggacgcctggatgggcactcaccctaagtatctagaaatgatggaattagatataggagatgccacccaagtttatgtagcgttcttggtttacctggacctcatggaaagcaaaagctggcatgaagtaaactgtgtaggattaccagaactccagctcatctgccttgttggtactgagatagaaggggaggggttacagactgtggtgcctacccccatcactgcttccctcagccataacaggataagggagatcttgaaggcatctcgaaagttgcaaggtgatccagatttgccgatgtcttttactttggccatagtggagtctgattctacaatagtctattataaacttactgatggatttatgctgccagaccctcagaatatttctcttagaaga

SEQ ID NO: 88 - protein, 171 aa, synthetic construct
MEERGDSEPTPGCSGLGPGGVRGFGDGGGAPSWAPEDAWMGTHPKYLEMMELDIGDATQVYVAFLVYLDLMESKSWHEVNCVGLPELQLICLVGTEIEGEGLQTVVPTPITASLSHNRIREILKASRKLQGDPDLPMSFTLAIVESDSTIVYYKLTDGFMLPDPQNISLRR

SEQ ID NO: 89 - DNA, 558 bp, synthetic construct
  source 1..558: mol_type = other DNA
ggtggtggcacccctaaggctcccaacctggagcctccactcccagaagaggaaaaggagggcagcgacctgagaccagtggtcatcgatgggagcaacgtggccatgagccatgggaacaaggaggtcttctcctgccggggcatcctgctggcagtgaactggtttctggagcggggccacacagacatcacagtgtttgtgccatcctggaggaaggagcagcctcggcccgacgtgcccatcacagaccagcacatcctgcgggaactggagaagaagaagatcctggtgttcacaccatcacgacgcgtgggtggcaagcgggtggtgtgctatgacgacagattcattgtgaagctggcctacgagtctgacgggatcgtggtttccaacgacacataccgtgacctccaaggcgagcggcaggagtggaagcgcttcatcgaggagcggctgctcatgtactccttcgtcaatgacaagtttatgccccctgatgacccactgggccggcacgggcccagcctggacaacttcctgcgtaagaagccactc

SEQ ID NO: 90 - protein, 186 aa, synthetic construct
GGGTPKAPNLEPPLPEEEKEGSDLRPVVIDGSNVAMSHGNKEVFSCRGILLAVNWFLERGHTDITVFVPSWRKEQPRPDVPITDQHILRELEKKKILVFTPSRRVGGKRVVCYDDRFIVKLAYESDGIVVSNDTYRDLQGERQEWKRFIEERLLMYSFVNDKFMPPDDPLGRHGPSLDNFLRKKPL

SEQ ID NO: 91 - protein, 16 aa, synthetic construct
SGSETPGTSESATPES

SEQ ID NO: 92 - protein, 5 aa, synthetic construct
GGGGS

SEQ ID NO: 93 - DNA, 42 bp, synthetic construct
  source 1..42: mol_type = other DNA
ctgctgctgctgctgctgctgctgctgctgctgctgctgctg

SEQ ID NO: 94 - DNA, 767 bp, synthetic construct
  source 1..767: mol_type = other DNA
atggtgagcaagggcgaggaggataacatggccatcatcaaggagttcatgcgcttcaaggtgcacatggagggctccgtgaacggccacgagttcgagatcgagggcgagggcgagggccgcccctacgagggcacccagaccgccaagctgaaggtgaccaagggtggccccctgcccttcgcctgggacatcctgtcccctcagttcatgtacggctccaaggcctacgtgaagcaccccgccgacatccccgactacttgaagctgtccttccccgagggcttcaagtgggagcgcgtgatgaacttcgaggacggcggcgtggtgaccgtgacccaggactcctccctgcaggacggcgagttcatctacaaggtgaagctgcgcggcaccaacttcccctccgacggccccgtaatgcagaagaagactatgggctgggaggcctcctccgagcggatgtaccccgaggacggcgccctgaagggcgagatcaagcagaggctgaagctgaaggacggcggccactacgacgctgaggtcaagaccacctacaaggccaagaagcccgtgcagctgcccggcgcctacaacgtcaacatcaagttggacatcacctcccacaacgaggactacaccatcgtggaacagtacgaacgcgccgagggccgccactccaccggcggcatggacgagctgtacaagtaggttgctagctgctgctgctgctgctgctgctgctgctgctgctgctgctgctcgag

SEQ ID NO: 95 - protein, 504 aa, synthetic construct
GRSRLLEDFRNNRYPNLQLREIAGHIMEFSQDQHGSRFIELKLERATPAERQLVFNEILQAAYQLMVDVFGNYVIQKFFEFGSLEQKLALAERIRGHVLSLALQMYGSYVIRKALEFIPSDQQNEMVRELDGHVLKCVKDQNGSYVVEKCIECVQPQSLQFIIDAFKGQVFALSTHPYGNRVIQRILEHCLPDQTLPILEELHQHTEQLVQDQYGSYVIRHVLEHGRPEDKSKIVAEIRGNVLVLSQHKFASNVVEKCVTHASRTERAVLIDEVCTMNDGPHSALYTMMKDQYANYVVQKMIDVAEPGQRKIVMHKIRPHIATLRKYTYGKHILAKLEKYYMKNGVDLGVDTGNGSQMVMGLGVLLLVFVLGLGLTPPTLAQDNSRYTHFLTQHYDAKPQGRDDRYCESIMRRRGLTSPCKDINTFIHGNKRSIKAICENKNGNPHRENLRISKSSFQVTTCKLHGGSPWPPCQYRATAGFRNVVVACENGLPVHLDQSIFRRP

SEQ ID NO: 96 - protein, 480 aa, synthetic construct
GRSRLLEDFRNNRYPNLQLREIAGHIMEFSQDQHGSRFIELKLERATPAERQLVFNEILQAAYQLMVDVFGNYVIQKFFEFGSLEQKLALAERIRGHVLSLALQMYGSYVIRKALEFIPSDQQNEMVRELDGHVLKCVKDQNGSYVVEKCIECVQPQSLQFIIDAFKGQVFALSTHPYGNRVIQRILEHCLPDQTLPILEELHQHTEQLVQDQYGSYVIRHVLEHGRPEDKSKIVAEIRGNVLVLSQHKFASNVVEKCVTHASRTERAVLIDEVCTMNDGPHSALYTMMKDQYANYVVQKMIDVAEPGQRKIVMHKIRPHIATLRKYTYGKHILAKLEKYYMKNGVDLGVDTGNGSQQDNSRYTHFLTQHYDAKPQGRDDRYCESIMRRRGLTSPCKDINTFIHGNKRSIKAICENKNGNPHRENLRISKSSFQVTTCKLHGGSPWPPCQYRATAGFRNVVVACENGLPVHLDQSIFRRP

SEQ ID NO: 97 - protein, 716 aa, synthetic construct
GRSRLLEDFRNNRYPNLQLREIAGHIMEFSQDQHGSRFIELKLERATPAERQLVFNEILQAAYQLMVDVFGNYVIQKFFEFGSLEQKLALAERIRGHVLSLALQMYGSYVIRKALEFIPSDQQNEMVRELDGHVLKCVKDQNGSYVVEKCIECVQPQSLQFIIDAFKGQVFALSTHPYGNRVIQRILEHCLPDQTLPILEELHQHTEQLVQDQYGSYVIRHVLEHGRPEDKSKIVAEIRGNVLVLSQHKFASNVVEKCVTHASRTERAVLIDEVCTMNDGPHSALYTMMKDQYANYVVQKMIDVAEPGQRKIVMHKIRPHIATLRKYTYGKHILAKLEKYYMKNGVDLGVDTGNGSQIDEKYKIADTSEGGIYLGFYEKQEVAVKTFCEGSPRAQREVSCLQSSRENSHLVTFYGSESHRGHLFVCVTLCEQTLEACLDVHRGEDVENEEDEFARNVLSSIFKAVQELHLSCGYTHQDLQPQNILIDSKKAAHLADFDKSIKWAGDPQEVKRDLEDLGRLVLYVVKKGSISFEDLKAQSNEEVVQLSPDEETKDLIHRLFHPGEHVRDCLSDLLGHPFFWTWESRYRTLRNVGNESDIKTRKSESEILRLLQPGPSEHSKSFDKWTTKINECVMKKMNKFYEKRGNFYQNTVGDLLKFIRNLGEHIDEEKHKKMKLKIGDPSLYFQKTFPDLVIYVYTKLQNTEYRKHFPQTHSPN

SEQ ID NO: 98 - protein, 476 aa, synthetic construct
GRSRLLEDFRNNRYPNLQLREIAGHIMEFSQDQHGSRFIELKLERATPAERQLVFNEILQAAYQLMVDVFGNYVIQKFFEFGSLEQKLALAERIRGHVLSLALQMYGSYVIRKALEFIPSDQQNEMVRELDGHVLKCVKDQNGSYVVEKCIECVQPQSLQFIIDAFKGQVFALSTHPYGNRVIQRILEHCLPDQTLPILEELHQHTEQLVQDQYGSYVIRHVLEHGRPEDKSKIVAEIRGNVLVLSQHKFASNVVEKCVTHASRTERAVLIDEVCTMNDGPHSALYTMMKDQYANYVVQKMIDVAEPGQRKIVMHKIRPHIATLRKYTYGKHILAKLEKYYMKNGVDLGVDTGNGSQHYLLPDTNVLLHQIDVLEDPAIRNVIVLQTVLQEVRNRSAPVYKRIRDVTNNQEKHFYTFTNEHHRETYVEQEQGENANDRNDRAIRVAAKWYNEHLKKMSADNQLQVIFITNDRRNKE

SEQ ID NO: 99 - protein, 485 aa, synthetic construct
GRSRLLEDFRNNRYPNLQLREIAGHIMEFSQDQHGSRFIELKLERATPAERQLVFNEILQAAYQLMVDVFGNYVIQKFFEFGSLEQKLALAERIRGHVLSLALQMYGSYVIRKALEFIPSDQQNEMVRELDGHVLKCVKDQNGSYVVEKCIECVQPQSLQFIIDAFKGQVFALSTHPYGNRVIQRILEHCLPDQTLPILEELHQHTEQLVQDQYGSYVIRHVLEHGRPEDKSKIVAEIRGNVLVLSQHKFASNVVEKCVTHASRTERAVLIDEVCTMNDGPHSALYTMMKDQYANYVVQKMIDVAEPGQRKIVMHKIRPHIATLRKYTYGKHILAKLEKYYMKNGVDLGVDTGNGSQKESRAKKFQRQHMDSDSSPSSSSTYCNQMMRRRNMTQGRCKPVNTFVHEPLVDVQNVCFQEKVTCKNGQGNCYKSNSSMHITDCRLTNGSRYPNCAYRTSPKERHIIVACEGSPYVPVHFDASVEDST

SEQ ID NO: 100 - protein, 916 aa, synthetic construct
GRSRLLEDFRNNRYPNLQLREIAGHIMEFSQDQHGSRFIELKLERATPAERQLVFNEILQAAYQLMVDVFGNYVIQKFFEFGSLEQKLALAERIRGHVLSLALQMYGSYVIRKALEFIPSDQQNEMVRELDGHVLKCVKDQNGSYVVEKCIECVQPQSLQFIIDAFKGQVFALSTHPYGNRVIQRILEHCLPDQTLPILEELHQHTEQLVQDQYGSYVIRHVLEHGRPEDKSKIVAEIRGNVLVLSQHKFASNVVEKCVTHASRTERAVLIDEVCTMNDGPHSALYTMMKDQYANYVVQKMIDVAEPGQRKIVMHKIRPHIATLRKYTYGKHILAKLEKYYMKNGVDLGVDTGNGSQAVAVDLGNRKLEISSGKLARFADGSAVVQSGDTAVMVTAVSKTKPSPSQFMPLVVDYRQKAAAAGRIPTNYLRREIGTSDKEILTSRIIDRSIRPLFPAGYFYDTQVLCNLLAVDGVNEPDVLAINGASVALSLSDIPWNGPVGAVRIGIIDGEYVVNPTRKEMSSSTLNLVVAGAPKSQIVMLEASAENILQQDFCHAIKVGVKYTQQIIQGIQQLVKETGVTKRTPQKLFTPSPEIVKYTHKLAMERLYAVFTDYEHDKVSRDEAVNKIRLDTEEQLKEKFPEADPYEIIESFNVVAKEVFRSIVLNEYKRCDGRDLTSLRNVSCEVDMFKTLHGSALFQRGQTQVLCTVTFDSLESGIKSDQVITAINGIKDKNFMLHYEFPPYATNEIGKVTGLNRRELGHGALAEKALYPVIPRDFPFTIRVTSEVLESNGSSSMASACGGSLALMDSGVPISSAVAGVAIGLVTKTDPEKGEIEDYRLLTDILGIEDYNGDMDFKIAGTNKGITALQADIKLPGIPIKIVMEAIQQASVAKKEILQIMNKTISKPRASRKENG

SEQ ID NO: 101 - protein, 522 aa, synthetic construct
GRSRLLEDFRNNRYPNLQLREIAGHIMEFSQDQHGSRFIELKLERATPAERQLVFNEILQAAYQLMVDVFGNYVIQKFFEFGSLEQKLALAERIRGHVLSLALQMYGSYVIRKALEFIPSDQQNEMVRELDGHVLKCVKDQNGSYVVEKCIECVQPQSLQFIIDAFKGQVFALSTHPYGNRVIQRILEHCLPDQTLPILEELHQHTEQLVQDQYGSYVIRHVLEHGRPEDKSKIVAEIRGNVLVLSQHKFASNVVEKCVTHASRTERAVLIDEVCTMNDGPHSALYTMMKDQYANYVVQKMIDVAEPGQRKIVMHKIRPHIATLRKYTYGKHILAKLEKYYMKNGVDLGVDTGNGSQMVWVDLEMTGLDIEKDQIIEMACLITDSDLNILAEGPNLIIKQPDELLDSMSDWCKEHHGKSGLTKAVKESTITLQQAEYEFLSFVRQQTPPGLCPLAGNSVHEDKKFLDKYMPQFMKHLHYRIIDVSTVKELCRRWYPEEYEFAPKKAASHRALDDISESIKEL

SEQ ID NO: 102 - protein, 500 aa, synthetic construct
GRSRLLEDFRNNRYPNLQLREIAGHIMEFSQDQHGSRFIELKLERATPAERQLVFNEILQAAYQLMVDVFGNYVIQKFFEFGSLEQKLALAERIRGHVLSLALQMYGSYVIRKALEFIPSDQQNEMVRELDGHVLKCVKDQNGSYVVEKCIECVQPQSLQFIIDAFKGQVFALSTHPYGNRVIQRILEHCLPDQTLPILEELHQHTEQLVQDQYGSYVIRHVLEHGRPEDKSKIVAEIRGNVLVLSQHKFASNVVEKCVTHASRTERAVLIDEVCTMNDGPHSALYTMMKDQYANYVVQKMIDVAEPGQRKIVMHKIRPHIATLRKYTYGKHILAKLEKYYMKNGVDLGVDTGNGSQDLLKTAFVNSCYIKSEEAKRQQLGIEKEAVLLNLKSNQELSEQGTSFSQTCLTQFLEDEYPDMPTEGIKNLVDFLTGEEVVCHVARNLAVEQLTLSEEFPVPPAVLQQTFFAVIGALLQSSGPERTALFIRDFLITQMTGKEL

SEQ ID NO: 103 - protein, 645 aa, synthetic construct
GRSRLLEDFRNNRYPNLQLREIAGHIMEFSQDQHGSRFIELKLERATPAERQLVFNEILQAAYQLMVDVFGNYVIQKFFEFGSLEQKLALAERIRGHVLSLALQMYGSYVIRKALEFIPSDQQNEMVRELDGHVLKCVKDQNGSYVVEKCIECVQPQSLQFIIDAFKGQVFALSTHPYGNRVIQRILEHCLPDQTLPILEELHQHTEQLVQDQYGSYVIRHVLEHGRPEDKSKIVAEIRGNVLVLSQHKFASNVVEKCVTHASRTERAVLIDEVCTMNDGPHSALYTMMKDQYANYVVQKMIDVAEPGQRKIVMHKIRPHIATLRKYTYGKHILAKLEKYYMKNGVDLGVDTGNGSQMAAVLQRVERLSNRVVRVLGCNPGPMTLQGTNTYLVGTGPRRILIDTGEPAIPEYISCLKQALTEFNTAIQEIVVTHWHRDHSGGIGDICKSINNDTTYCIKKLPRNPQREEIIGNGEQQYVYLKDGDVIKTEGATLRVLYTPGHTDDHMALLLEEENAIFSGDCILGEGTTVFEDLYDYMNSLKELLKIKADIIYPGHGPVIHNAEAKIQQYISHRNIREQQILTLFRENFEKSFTVMELVKIIYKNTPENLHEMAKHNLLLHLKKLEKEGKIFSNTDPDKKWKAHL

SEQ ID NO: 104 - protein, 528 aa, synthetic construct
GRSRLLEDFRNNRYPNLQLREIAGHIMEFSQDQHGSRFIELKLERATPAERQLVFNEILQAAYQLMVDVFGNYVIQKFFEFGSLEQKLALAERIRGHVLSLALQMYGSYVIRKALEFIPSDQQNEMVRELDGHVLKCVKDQNGSYVVEKCIECVQPQSLQFIIDAFKGQVFALSTHPYGNRVIQRILEHCLPDQTLPILEELHQHTEQLVQDQYGSYVIRHVLEHGRPEDKSKIVAEIRGNVLVLSQHKFASNVVEKCVTHASRTERAVLIDEVCTMNDGPHSALYTMMKDQYANYVVQKMIDVAEPGQRKIVMHKIRPHIATLRKYTYGKHILAKLEKYYMKNGVDLGVDTGNGSQMEERGDSEPTPGCSGLGPGGVRGFGDGGGAPSWAPEDAWMGTHPKYLEMMELDIGDATQVYVAFLVYLDLMESKSWHEVNCVGLPELQLICLVGTEIEGEGLQTVVPTPITASLSHNRIREILKASRKLQGDPDLPMSFTLAIVESDSTIVYYKLTDGFMLPDPQNISLRR

SEQ ID NO: 105 - protein, 543 aa, synthetic construct
GRSRLLEDFRNNRYPNLQLREIAGHIMEFSQDQHGSRFIELKLERATPAERQLVFNEILQAAYQLMVDVFGNYVIQKFFEFGSLEQKLALAERIRGHVLSLALQMYGSYVIRKALEFIPSDQQNEMVRELDGHVLKCVKDQNGSYVVEKCIECVQPQSLQFIIDAFKGQVFALSTHPYGNRVIQRILEHCLPDQTLPILEELHQHTEQLVQDQYGSYVIRHVLEHGRPEDKSKIVAEIRGNVLVLSQHKFASNVVEKCVTHASRTERAVLIDEVCTMNDGPHSALYTMMKDQYANYVVQKMIDVAEPGQRKIVMHKIRPHIATLRKYTYGKHILAKLEKYYMKNGVDLGVDTGNGSQGGGTPKAPNLEPPLPEEEKEGSDLRPVVIDGSNVAMSHGNKEVFSCRGILLAVNWFLERGHTDITVFVPSWRKEQPRPDVPITDQHILRELEKKKILVFTPSRRVGGKRVVCYDDRFIVKLAYESDGIVVSNDTYRDLQGERQEWKRFIEERLLMYSFVNDKFMPPDDPLGRHGPSLDNFLRKKPL

SEQ ID NO: 106 - protein, 504 aa, synthetic construct
MVMGLGVLLLVFVLGLGLTPPTLAQDNSRYTHFLTQHYDAKPQGRDDRYCESIMRRRGLTSPCKDINTFIHGNKRSIKAICENKNGNPHRENLRISKSSFQVTTCKLHGGSPWPPCQYRATAGFRNVVVACENGLPVHLDQSIFRRPVDTGNGSQGRSRLLEDFRNNRYPNLQLREIAGHIMEFSQDQHGSRFIELKLERATPAERQLVFNEILQAAYQLMVDVFGNYVIQKFFEFGSLEQKLALAERIRGHVLSLALQMYGSYVIRKALEFIPSDQQNEMVRELDGHVLKCVKDQNGSYVVEKCIECVQPQSLQFIIDAFKGQVFALSTHPYGNRVIQRILEHCLPDQTLPILEELHQHTEQLVQDQYGSYVIRHVLEHGRPEDKSKIVAEIRGNVLVLSQHKFASNVVEKCVTHASRTERAVLIDEVCTMNDGPHSALYTMMKDQYANYVVQKMIDVAEPGQRKIVMHKIRPHIATLRKYTYGKHILAKLEKYYMKNGVDLG

SEQ ID NO: 107 - protein, 480 aa, synthetic construct
QDNSRYTHFLTQHYDAKPQGRDDRYCESIMRRRGLTSPCKDINTFIHGNKRSIKAICENKNGNPHRENLRISKSSFQVTTCKLHGGSPWPPCQYRATAGFRNVVVACENGLPVHLDQSIFRRPVDTGNGSQGRSRLLEDFRNNRYPNLQLREIAGHIMEFSQDQHGSRFIELKLERATPAERQLVFNEILQAAYQLMVDVFGNYVIQKFFEFGSLEQKLALAERIRGHVLSLALQMYGSYVIRKALEFIPSDQQNEMVRELDGHVLKCVKDQNGSYVVEKCIECVQPQSLQFIIDAFKGQVFALSTHPYGNRVIQRILEHCLPDQTLPILEELHQHTEQLVQDQYGSYVIRHVLEHGRPEDKSKIVAEIRGNVLVLSQHKFASNVVEKCVTHASRTERAVLIDEVCTMNDGPHSALYTMMKDQYANYVVQKMIDVAEPGQRKIVMHKIRPHIATLRKYTYGKHILAKLEKYYMKNGVDLG

SEQ ID NO: 108 - protein, 485 aa, synthetic construct
KESRAKKFQRQHMDSDSSPSSSSTYCNQMMRRRNMTQGRCKPVNTFVHEPLVDVQNVCFQEKVTCKNGQGNCYKSNSSMHITDCRLTNGSRYPNCAYRTSPKERHIIVACEGSPYVPVHFDASVEDSTVDTGNGSQGRSRLLEDFRNNRYPNLQLREIAGHIMEFSQDQHGSRFIELKLERATPAERQLVFNEILQAAYQLMVDVFGNYVIQKFFEFGSLEQKLALAERIRGHVLSLALQMYGSYVIRKALEFIPSDQQNEMVRELDGHVLKCVKDQNGSYVVEKCIECVQPQSLQFIIDAFKGQVFALSTHPYGNRVIQRILEHCLPDQTLPILEELHQHTEQLVQDQYGSYVIRHVLEHGRPEDKSKIVAEIRGNVLVLSQHKFASNVVEKCVTHASRTERAVLIDEVCTMNDGPHSALYTMMKDQYANYVVQKMIDVAEPGQRKIVMHKIRPHIATLRKYTYGKHILAKLEKYYMKNGVDLG

SEQ ID NO: 109 - protein, 916 aa, synthetic construct
AVAVDLGNRKLEISSGKLARFADGSAVVQSGDTAVMVTAVSKTKPSPSQFMPLVVDYRQKAAAAGRIPTNYLRREIGTSDKEILTSRIIDRSIRPLFPAGYFYDTQVLCNLLAVDGVNEPDVLAINGASVALSLSDIPWNGPVGAVRIGIIDGEYVVNPTRKEMSSSTLNLVVAGAPKSQIVMLEASAENILQQDFCHAIKVGVKYTQQIIQGIQQLVKETGVTKRTPQKLFTPSPEIVKYTHKLAMERLYAVFTDYEHDKVSRDEAVNKIRLDTEEQLKEKFPEADPYEIIESFNVVAKEVFRSIVLNEYKRCDGRDLTSLRNVSCEVDMFKTLHGSALFQRGQTQVLCTVTFDSLESGIKSDQVITAINGIKDKNFMLHYEFPPYATNEIGKVTGLNRRELGHGALAEKALYPVIPRDFPFTIRVTSEVLESNGSSSMASACGGSLALMDSGVPISSAVAGVAIGLVTKTDPEKGEIEDYRLLTDILGIEDYNGDMDFKIAGTNKGITALQADIKLPGIPIKIVMEAIQQASVAKKEILQIMNKTISKPRASRKENGVDTGNGSQGRSRLLEDFRNNRYPNLQLREIAGHIMEFSQDQHGSRFIELKLERATPAERQLVFNEILQAAYQLMVDVFGNYVIQKFFEFGSLEQKLALAERIRGHVLSLALQMYGSYVIRKALEFIPSDQQNEMVRELDGHVLKCVKDQNGSYVVEKCIECVQPQSLQFIIDAFKGQVFALSTHPYGNRVIQRILEHCLPDQTLPILEELHQHTEQLVQDQYGSYVIRHVLEHGRPEDKSKIVAEIRGNVLVLSQHKFASNVVEKCVTHASRTERAVLIDEVCTMNDGPHSALYTMMKDQYANYVVQKMIDVAEPGQRKIVMHKIRPHIATLRKYTYGKHILAKLEKYYMKNGVDLG

SEQ ID NO: 110 - protein, 522 aa, synthetic construct
MVWVDLEMTGLDIEKDQIIEMACLITDSDLNILAEGPNLIIKQPDELLDSMSDWCKEHHGKSGLTKAVKESTITLQQAEYEFLSFVRQQTPPGLCPLAGNSVHEDKKFLDKYMPQFMKHLHYRIIDVSTVKELCRRWYPEEYEFAPKKAASHRALDDISESIKELVDTGNGSQGRSRLLEDFRNNRYPNLQLREIAGHIMEFSQDQHGSRFIELKLERATPAERQLVFNEILQAAYQLMVDVFGNYVIQKFFEFGSLEQKLALAERIRGHVLSLALQMYGSYVIRKALEFIPSDQQNEMVRELDGHVLKCVKDQNGSYVVEKCIECVQPQSLQFIIDAFKGQVFALSTHPYGNRVIQRILEHCLPDQTLPILEELHQHTEQLVQDQYGSYVIRHVLEHGRPEDKSKIVAEIRGNVLVLSQHKFASNVVEKCVTHASRTERAVLIDEVCTMNDGPHSALYTMMKDQYANYVVQKMIDVAEPGQRKIVMHKIRPHIATLRKYTYGKHILAKLEKYYMKNGVDLG

SEQ ID NO: 111 - protein, 543 aa, synthetic construct
GGGTPKAPNLEPPLPEEEKEGSDLRPVVIDGSNVAMSHGNKEVFSCRGILLAVNWFLERGHTDITVFVPSWRKEQPRPDVPITDQHILRELEKKKILVFTPSRRVGGKRVVCYDDRFIVKLAYESDGIVVSNDTYRDLQGERQEWKRFIEERLLMYSFVNDKFMPPDDPLGRHGPSLDNFLRKKPLVDTGNGSQGRSRLLEDFRNNRYPNLQLREIAGHIMEFSQDQHGSRFIELKLERATPAERQLVFNEILQAAYQLMVDVFGNYVIQKFFEFGSLEQKLALAERIRGHVLSLALQMYGSYVIRKALEFIPSDQQNEMVRELDGHVLKCVKDQNGSYVVEKCIECVQPQSLQFIIDAFKGQVFALSTHPYGNRVIQRILEHCLPDQTLPILEELHQHTEQLVQDQYGSYVIRHVLEHGRPEDKSKIVAEIRGNVLVLSQHKFASNVVEKCVTHASRTERAVLIDEVCTMNDGPHSALYTMMKDQYANYVVQKMIDVAEPGQRKIVMHKIRPHIATLRKYTYGKHILAKLEKYYMKNGVDLG

SEQ ID NO: 112 - DNA, 768 bp, synthetic construct
  source 1..768: mol_type = other DNA
atgcgccctgcagccctgcgcggggccctgctgggctgcctctgcctggcgttgctttgcctgggcggtgcggacaagcgcctgcgtgacaaccatgagtggaaaaaactaattatggttcagcactggcctgagacagtatgcgagaaaattcaaaacgactgtagagaccctccggattactggacaatacatggactatggcccgataaaagtgaaggatgtaatagatcgtggcccttcaatttagaagagattaaggatcttttgccagaaatgagggcatactggcctgacgtaattcactcgtttcccaatcgcagccgcttctggaagcatgagtgggaaaagcatgggacctgcgccgcccaggtggatgcgctcaactcccagaagaagtactttggcagaagcctggaactctacagggagctggacctcaacagtgtgcttctaaaattggggataaaaccatccatcaattactaccaagttgcagattttaaagatgcccttgccagagtatatggagtgatacccaaaatccagtgccttccaccaagccaggatgaggaagtacagacaattggtcagatagaactgtgcctcactaagcaagaccagcagctgcaaaactgcaccgagccgggggagcagccgtcccccaagcaggaagtctggctggcaaatggggccgccgagagccggggtctgagagtctgtgaagatggcccagtcttctatcccccacctaaaaagaccaagcat

SEQ ID NO: 113 - protein, 256 aa, synthetic construct
MRPAALRGALLGCLCLALLCLGGADKRLRDNHEWKKLIMVQHWPETVCEKIQNDCRDPPDYWTIHGLWPDKSEGCNRSWPFNLEEIKDLLPEMRAYWPDVIHSFPNRSRFWKHEWEKHGTCAAQVDALNSQKKYFGRSLELYRELDLNSVLLKLGIKPSINYYQVADFKDALARVYGVIPKIQCLPPSQDEEVQTIGQIELCLTKQDQQLQNCTEPGEQPSPKQEVWLANGAAESRGLRVCEDGPVFYPPPKKTKH

SEQ ID NO: 114 - DNA, 2358 bp, synthetic construct
  source 1..2358: mol_type = other DNA
atgtccttctcccgtgccctattgtgggctcggctcccggcggggcgccaggctggccaccgggcagccatctgctctgcccttcgtccccactttgggccctttcccggggttctggggcaagtttctgtccttgccaccgcctcctcctctgcctccggtggctccaaaataccaaacacgtccttgttcgtgcccctgactgtgaaacctcagggccccagcgccgacggcgacgtcggggccgagctaacccggcctctggacaagaatgaagtaaagaaggtcttagacaaattttacaagaggaaagaaattcagaaactgggtgctgattatggacttgatgctcgtctcttccaccaagctttcataagctttagaaattatattatgcagtctcattccctggatgtggacattcacattgttttgaatgatatttgcttcggtgcagctcatgcggatgatttattcccatttttcttgagacatgccaaacaaatatttcctgtgttggactgtaaggatgatctacgtaaaatcagtgacttaagaataccacctaactggtacccagatgctagagccatgcagcggaagataatatttcattcaggccccacaaacagtggaaagacttatcacgcaatccagaaatacttctcagcaaagtctggagtgtattgtggccctctaaaattactggcacatgagatcttcgaaaagagtaatgctgctggtgtgccatgtgacttggtgacaggtgaagagcgtgtgacagttcagccaaatgggaaacaggcttcacatgtttcttgtacagttgagatgtgcagtgttacaactccttatgaagtggctgtaattgatgaaattcaaatgattagagatccagccagaggatgggcctggaccagagcacttctaggactgtgtgctgaagaggttcatttgtgtggagaacctgctgctattgacctggtgatggagcttatgtacacaacgggggaggaagtggaggttcgagactataagaggcttacccccatttctgtgctggaccatgcactagaatctttagataaccttcggcctggggactgcattgtctgttttagcaagaatgatatttattctgtgagtcggcagattgaaattcggggattagaatcagctgttatatatggcagtctcccacctgggaccaaacttgctcaagcaaaaaagtttaatgatcccaatgacccatgcaaaatcttggttgctacagatgcaattggcatgggacttaatttgagcataaggagaattattttttactcccttataaagcccagtatcaatgaaaagggagagagagaactagaaccaatcacaacctctcaagccctgcagattgctggcagagctggcagattcagctcacggtttaaagaaggagaggttacaacaatgaatcatgaagatctcagtttattaaaggaaattttgaagaggcctgtggatcctataagggcagctggtcttcatccaactgctgagcagattgaaatgtttgcctaccatctccctgatgcaacactgtccaatctcattgatatttttgtagacttttcacaagttgatgggcagtattttgtctgcaatatggatgattttaaattttctgcagagttgatccagcatattccactaagtctgcgagtgaggtatgttttctgcacagctcctatcaacaagaagcagccttttgtgtgttcttcactgttacagtttgccaggcagtatagcaggaatgagcccctgacctttgcatggttacgccgatacatcaaatggcctttacttccacctaagaatattaaagacctcatggatcttgaagctgtccacgatgtcttggatctttacttgtggctaagctaccgatttatggatatgtttccagatgccagccttattcgagatctccagaaagaactagatggtattatccaagatggtgtgcacaatatcactaaattgattaaaatgtctgagacgcataagctgttgaatttggagggctttccatcagggagccagtcacgattgtcaggaaccttaaagagccaagctagaaggacacgcggcaccaaagctctagggagtaaagctactgagccacccagccccgatgcaggagagctgtcccttgcttccagattggtgcagcaaggactcctcactccagacatgctgaaacagctagaaaaagagtggatgacacaacaaactgaacacaacaaagaaaaaacagagtctgggactcatccaaaagggacgagaagaaagaagaaggaacctgattcggac

SEQ ID NO: 115 - protein, 786 aa, synthetic construct
MSFSRALLWARLPAGRQAGHRAAICSALRPHFGPFPGVLGQVSVLATASSSASGGSKIPNTSLFVPLTVKPQGPSADGDVGAELTRPLDKNEVKKVLDKFYKRKEIQKLGADYGLDARLFHQAFISFRNYIMQSHSLDVDIHIVLNDICFGAAHADDLFPFFLRHAKQIFPVLDCKDDLRKISDLRIPPNWYPDARAMQRKIIFHSGPTNSGKTYHAIQKYFSAKSGVYCGPLKLLAHEIFEKSNAAGVPCDLVTGEERVTVQPNGKQASHVSCTVEMCSVTTPYEVAVIDEIQMIRDPARGWAWTRALLGLCAEEVHLCGEPAAIDLVMELMYTTGEEVEVRDYKRLTPISVLDHALESLDNLRPGDCIVCFSKNDIYSVSRQIEIRGLESAVIYGSLPPGTKLAQAKKFNDPNDPCKILVATDAIGMGLNLSIRRIIFYSLIKPSINEKGERELEPITTSQALQIAGRAGRFSSRFKEGEVTTMNHEDLSLLKEILKRPVDPIRAAGLHPTAEQIEMFAYHLPDATLSNLIDIFVDFSQVDGQYFVCNMDDFKFSAELIQHIPLSLRVRYVFCTAPINKKQPFVCSSLLQFARQYSRNEPLTFAWLRRYIKWPLLPPKNIKDLMDLEAVHDVLDLYLWLSYRFMDMFPDASLIRDLQKELDGIIQDGVHNITKLIKMSETHKLLNLEGFPSGSQSRLSGTLKSQARRTRGTKALGSKATEPPSPDAGELSLASRLVQQGLLTPDMLKQLEKEWMTQQTEHNKEKTESGTHPKGTRRKKKEPDSD

SEQ ID NO: 116 - protein, 589 aa, synthetic construct
GRSRLLEDFRNNRYPNLQLREIAGHIMEFSQDQHGSRFIELKLERATPAERQLVFNEILQAAYQLMVDVFGNYVIQKFFEFGSLEQKLALAERIRGHVLSLALQMYGSYVIRKALEFIPSDQQNEMVRELDGHVLKCVKDQNGSYVVEKCIECVQPQSLQFIIDAFKGQVFALSTHPYGNRVIQRILEHCLPDQTLPILEELHQHTEQLVQDQYGSYVIRHVLEHGRPEDKSKIVAEIRGNVLVLSQHKFASNVVEKCVTHASRTERAVLIDEVCTMNDGPHSALYTMMKDQYANYVVQKMIDVAEPGQRKIVMHKIRPHIATLRKYTYGKHILAKLEKYYMKNGVDLGVEEHRRSTDKRLRDNHEWKKLIMVQHWPETVCEKIQNDCRDPPDYWTIHGLWPDKSEGCNRSWPFNLEEIKDLLPEMRAYWPDVIHSFPNRSRFWKHEWEKHGTCAAQVDALNSQKKYFGRSLELYRELDLNSVLLKLGIKPSINYYQVADFKDALARVYGVIPKIQCLPPSQDEEVQTIGQIELCLTKQDQQLQNCTEPGEQPSPKQEVWLANGAAESRGLRVCEDGPVFYPPPKKTKH

SEQ ID NO: 117 - protein, 589 aa, synthetic construct
DKRLRDNHEWKKLIMVQHWPETVCEKIQNDCRDPPDYWTIHGLWPDKSEGCNRSWPFNLEEIKDLLPEMRAYWPDVIHSFPNRSRFWKHEWEKHGTCAAQVDALNSQKKYFGRSLELYRELDLNSVLLKLGIKPSINYYQVADFKDALARVYGVIPKIQCLPPSQDEEVQTIGQIELCLTKQDQQLQNCTEPGEQPSPKQEVWLANGAAESRGLRVCEDGPVFYPPPKKTKHVEEHRRSTGRSRLLEDFRNNRYPNLQLREIAGHIMEFSQDQHGSRFIELKLERATPAERQLVFNEILQAAYQLMVDVFGNYVIQKFFEFGSLEQKLALAERIRGHVLSLALQMYGSYVIRKALEFIPSDQQNEMVRELDGHVLKCVKDQNGSYVVEKCIECVQPQSLQFIIDAFKGQVFALSTHPYGNRVIQRILEHCLPDQTLPILEELHQHTEQLVQDQYGSYVIRHVLEHGRPEDKSKIVAEIRGNVLVLSQHKFASNVVEKCVTHASRTERAVLIDEVCTMNDGPHSALYTMMKDQYANYVVQKMIDVAEPGQRKIVMHKIRPHIATLRKYTYGKHILAKLEKYYMKNGVDLG

SEQ ID NO: 118 - protein, 523 aa, synthetic construct
GRSRLLEDFRNNRYPNLQLREIAGHIMEFSQDQHGSRFIELKLERATPAERQLVFNEILQAAYQLMVDVFGNYVIQKFFEFGSLEQKLALAERIRGHVLSLALQMYGSYVIRKALEFIPSDQQNEMVRELDGHVLKCVKDQNGSYVVEKCIECVQPQSLQFIIDAFKGQVFALSTHPYGNRVIQRILEHCLPDQTLPILEELHQHTEQLVQDQYGSYVIRHVLEHGRPEDKSKIVAEIRGNVLVLSQHKFASNVVEKCVTHASRTERAVLIDEVCTMNDGPHSALYTMMKDQYANYVVQKMIDVAEPGQRKIVMHKIRPHIATLRKYTYGKHILAKLEKYYMKNGVDLGVEEHRRSTVLDHALESLDNLRPGDCIVCFSKNDIYSVSRQIEIRGLESAVIYGSLPPGTKLAQAKKFNDPNDPCKILVATDAIGMGLNLSIRRIIFYSLIKPSINEKGERELEPITTSQALQIAGRAGRFSSRFKEGEVTTMNHEDLSLLKEILKRPVDPIRAAGLHPTAEQIE

SEQ ID NO: 119 - DNA, 318 bp, synthetic construct
  misc_feature 7: note = n is a, c, g, or t
  misc_feature 16: note = n is a, c, g, or t
  misc_feature 38: note = n is a, c, g, or t
  misc_feature 40: note = n is a, c, g, or t
  misc_feature 52: note = n is a, c, g, or t
  misc_feature 60: note = n is a, c, g, or t
  misc_feature 83: note = n is a, c, g, or t
  misc_feature 111..112: note = n is a, c, g, or t
  misc_feature 115: note = n is a, c, g, or t
  misc_feature 134: note = n is a, c, g, or t
  misc_feature 143: note = n is a, c, g, or t
  misc_feature 170: note = n is a, c, g, or t
  misc_feature 183: note = n is a, c, g, or t
  misc_feature 205: note = n is a, c, g, or t
  misc_feature 237: note = n is a, c, g, or t
  misc_feature 245: note = n is a, c, g, or t
  misc_feature 265: note = n is a, c, g, or t
  misc_feature 279: note = n is a, c, g, or t
  misc_feature 314: note = n is a, c, g, or t
  source 1..318: mol_type = other DNA
vdhasdnrgdcvcskndysvsrrgsavygsgtkaakkndndckvatdagmgnsrrysksnkgrttsaagragrssrkgvttmnhdskkrvdraaghtavhrrstgrsrdrnnrynraghmsdhgsrkratarvnaaymvdvgnyvkgskaarrghvsamygsyvrkasdnmvrdghvkcvkdngsyvvkccvsdakgvasthygnrvrhcdthhtvdygsyvrhvhgrdkskvargnvvshkasnvvkcvthasrtravdvctmndghsaytmmkdyanyvvkmdvagrkvmhkrhatrkytygkhakkyymkngvdg

SEQ ID NO: 120 - protein, 349 aa, Abies grandis; identical to SEQ ID NO: 1